European Patent Specification EP 2 970 407 B1, published November 15, 2023. Title: VARIANTS OF TISSUE INHIBITOR OF METALLOPROTEINASE TYPE THREE (TIMP-3), COMPOSITIONS AND METHODS. Applicant: AMGEN INC. The sequence listing filed with the application follows.

SEQUENCE LISTING (99 sequences)

SEQ ID NO: 1 - DNA, 633 bp, Homo sapiens
atgaccccttggctcgggctcatcgtgctcctgggcagctggagcctgggggactggggcgccgaggcgtgcacatgctcgcccagccacccccaggacgccttctgcaactccgacatcgtgatccgggccaaggtggtggggaagaagctggtaaaggaggggcccttcggcacgctggtctacaccatcaagcagatgaagatgtaccgaggcttcaccaagatgccccatgtgcagtacatccacacggaagcttccgagagtctctgtggccttaagctggaggtcaacaagtaccagtacctgctgacaggtcgcgtctatgatggcaagatgtacacggggctgtgcaacttcgtggagaggtgggaccagctcaccctctcccagcgcaaggggctgaactatcggtatcacctgggttgtaactgcaagatcaagtcctgctactacctgccttgctttgtgacttccaagaacgagtgtctctggaccgacatgctctccaatttcggttaccctggctaccagtccaaacactacgcctgcatccggcagaagggcggctactgcagctggtaccgaggatgggcccccccggataaaagcatcatcaatgccacagacccc

SEQ ID NO: 2 - protein, 211 aa, Homo sapiens
MTPWLGLIVLLGSWSLGDWGAEACTCSPSHPQDAFCNSDIVIRAKVVGKKLVKEGPFGTLVYTIKQMKMYRGFTKMPHVQYIHTEASESLCGLKLEVNKYQYLLTGRVYDGKMYTGLCNFVERWDQLTLSQRKGLNYRYHLGCNCKIKSCYYLPCFVTSKNECLWTDMLSNFGYPGYQSKHYACIRQKGGYCSWYRGWAPPDKSIINATDP

SEQ ID NO: 3 - protein, 211 aa, Artificial Sequence
  Description of Artificial Sequence: Synthetic polypeptide
  MOD_RES (1)..(1): Met or any amino acid from a heterologous signal peptide
  MOD_RES (2)..(2): Thr or any amino acid from a heterologous signal peptide
  MOD_RES (3)..(3): Pro or any amino acid from a heterologous signal peptide
  MOD_RES (4)..(4): Trp or any amino acid from a heterologous signal peptide
  MOD_RES (5)..(5): Leu or any amino acid from a heterologous signal peptide
  MOD_RES (6)..(6): Gly or any amino acid from a heterologous signal peptide
  MOD_RES (7)..(7): Leu or any amino acid from a heterologous signal peptide
  MOD_RES (8)..(8): Ile or any amino acid from a heterologous signal peptide
  MOD_RES (9)..(9): Val or any amino acid from a heterologous signal peptide
  MOD_RES (10)..(11): Leu or any amino acid from a heterologous signal peptide
  MOD_RES (12)..(12): Gly or any amino acid from a heterologous signal peptide
  MOD_RES (13)..(13): Ser or any amino acid from a heterologous signal peptide
  MOD_RES (14)..(14): Trp or any amino acid from a heterologous signal peptide
  MOD_RES (15)..(15): Ser or any amino acid from a heterologous signal peptide
  MOD_RES (16)..(16): Leu or any amino acid from a heterologous signal peptide
  MOD_RES (17)..(17): Gly or any amino acid from a heterologous signal peptide
  MOD_RES (18)..(18): Asp or any amino acid from a heterologous signal peptide
  MOD_RES (19)..(19): Trp or any amino acid from a heterologous signal peptide
  MOD_RES (20)..(20): Gly or any amino acid from a heterologous signal peptide
  MOD_RES (21)..(21): Ala or any amino acid from a heterologous signal peptide
  MOD_RES (22)..(22): Glu or any amino acid from a heterologous signal peptide
  MOD_RES (23)..(23): Ala or any amino acid from a heterologous signal peptide
  MOD_RES (45)..(45): Lys, Glu, Asn or Ser
  MOD_RES (47)..(47): Val or Thr
  MOD_RES (49)..(49): Lys, Glu, Asn or Ser
  MOD_RES (50)..(50): Lys or Asn
  MOD_RES (51)..(51): Leu, Asn or Thr
  MOD_RES (52)..(52): Val or Thr
  MOD_RES (53)..(53): Lys or Thr
  MOD_RES (56)..(56): Pro or Asn
  MOD_RES (57)..(57): Phe or Asn
  MOD_RES (58)..(58): Gly or Thr
  MOD_RES (63)..(63): Thr, Glu or Asn
  MOD_RES (65)..(65): Lys, Thr or Asn
  MOD_RES (67)..(67): Met or Thr
  MOD_RES (68)..(68): Lys or Ser
  MOD_RES (74)..(74): Thr or Glu
  MOD_RES (75)..(75): Lys or Asn
  MOD_RES (77)..(77): Pro or Thr
  MOD_RES (78)..(78): His, Asp, Glu or Asn
  MOD_RES (80)..(80): Gln, Glu or Thr
  MOD_RES (94)..(94): Lys or Asn
  MOD_RES (96)..(96): Glu, Thr or Asn
  MOD_RES (97)..(97): Val or Asn
  MOD_RES (98)..(98): Asn or Thr
  MOD_RES (99)..(99): Lys or Thr
  MOD_RES (110)..(110): Asp or Asn
  MOD_RES (112)..(112): Lys or Thr
  MOD_RES (126)..(126): Gln or Asn
  MOD_RES (133)..(133): Lys or Ser
  MOD_RES (138)..(138): Arg, Asn or Thr
  MOD_RES (140)..(140): His or Thr
  MOD_RES (158)..(158): Thr or Asn
  MOD_RES (160)..(160): Lys or Thr
  MOD_RES (166)..(166): Thr or Asn
  MOD_RES (168)..(168): Met or Thr
  MOD_RES (173)..(173): Gly or Thr
  MOD_RES (181)..(181): His or Asn
  MOD_RES (183)..(183): Ala or Thr
  MOD_RES (186)..(186): Arg or Asn
  MOD_RES (188)..(188): Lys or Thr
  MOD_RES (201)..(201): Pro or Asn
  MOD_RES (203)..(203): Lys or Thr
  MOD_RES (208)..(208): Ala, Val or Tyr
XXXXXXXXXXXXXXXXXXXXXXXCTCSPSHPQDAFCNSDIVIRAXVXGXXXXXEGXXXTLVYXIXQXXMYRGFXXMXXVXYIHTEASESLCGLXLXXXXYQYLLTGRVYXGXMYTGLCNFVERWDXLTLSQRXGLNYXYXLGCNCKIKSCYYLPCFVXSXNECLWXDXLSNFXYPGYQSKXYXCIXQXGGYCSWYRGWAPXDXSIINXTDP

SEQ ID NO: 4 - protein, 211 aa, Artificial Sequence
  Description of Artificial Sequence: Synthetic polypeptide
  MOD_RES (1)..(1): Met or any amino acid from a heterologous signal peptide
  MOD_RES (2)..(2): Thr or any amino acid from a heterologous signal peptide
  MOD_RES (3)..(3): Pro or any amino acid from a heterologous signal peptide
  MOD_RES (4)..(4): Trp or any amino acid from a heterologous signal peptide
  MOD_RES (5)..(5): Leu or any amino acid from a heterologous signal peptide
  MOD_RES (6)..(6): Gly or any amino acid from a heterologous signal peptide
  MOD_RES (7)..(7): Leu or any amino acid from a heterologous signal peptide
  MOD_RES (8)..(8): Ile or any amino acid from a heterologous signal peptide
  MOD_RES (9)..(9): Val or any amino acid from a heterologous signal peptide
  MOD_RES (10)..(11): Leu or any amino acid from a heterologous signal peptide
  MOD_RES (12)..(12): Gly or any amino acid from a heterologous signal peptide
  MOD_RES (13)..(13): Ser or any amino acid from a heterologous signal peptide
  MOD_RES (14)..(14): Trp or any amino acid from a heterologous signal peptide
  MOD_RES (15)..(15): Ser or any amino acid from a heterologous signal peptide
  MOD_RES (16)..(16): Leu or any amino acid from a heterologous signal peptide
  MOD_RES (17)..(17): Gly or any amino acid from a heterologous signal peptide
  MOD_RES (18)..(18): Asp or any amino acid from a heterologous signal peptide
  MOD_RES (19)..(19): Trp or any amino acid from a heterologous signal peptide
  MOD_RES (20)..(20): Gly or any amino acid from a heterologous signal peptide
  MOD_RES (21)..(21): Ala or any amino acid from a heterologous signal peptide
  MOD_RES (22)..(22): Glu or any amino acid from a heterologous signal peptide
  MOD_RES (23)..(23): Ala or any amino acid from a heterologous signal peptide
  MOD_RES (25)..(25): Thr, His, Lys, Pro, Arg, Ser or Trp
  MOD_RES (27)..(27): Ser or Ala
  MOD_RES (28)..(28): Pro, Asp, Leu or Ser
  MOD_RES (32)..(32): Gln or Asn
  MOD_RES (39)..(39): Asp or Thr
  MOD_RES (43)..(43): Arg, Thr, Phe, Ala or Asn
  MOD_RES (45)..(45): Lys, Ile or Thr
  MOD_RES (46)..(46): Val or Asp
  MOD_RES (48)..(48): Gly or Ser
  MOD_RES (49)..(49): Lys or Ser
  MOD_RES (51)..(51): Leu or Thr
  MOD_RES (53)..(53): Lys or Thr
  MOD_RES (54)..(54): Glu or Tyr
  MOD_RES (67)..(67): Met or Asn
  MOD_RES (68)..(68): Lys or Ile
  MOD_RES (78)..(78): His, Asp or Trp
  MOD_RES (202)..(202): Asp or Asn
  MOD_RES (207)..(207): Asn or Ser
XXXXXXXXXXXXXXXXXXXXXXXCXCXXSHPXDAFCNSXIVIXAXXVXXKXVXXGPFGTLVYTIKQXXMYRGFTKMPXVQYIHTEASESLCGLKLEVNKYQYLLTGRVYDGKMYTGLCNFVERWDQLTLSQRKGLNYRYHLGCNCKIKSCYYLPCFVTSKNECLWTDMLSNFGYPGYQSKHYACIRQKGGYCSWYRGWAPPXKSIIXATDP

SEQ ID NO: 5 - protein, 211 aa, Artificial Sequence
  Description of Artificial Sequence: Synthetic polypeptide
  MOD_RES (1)..(1): Met or any amino acid from a heterologous signal peptide
  MOD_RES (2)..(2): Thr or any amino acid from a heterologous signal peptide
  MOD_RES (3)..(3): Pro or any amino acid from a heterologous signal peptide
  MOD_RES (4)..(4): Trp or any amino acid from a heterologous signal peptide
  MOD_RES (5)..(5): Leu or any amino acid from a heterologous signal peptide
  MOD_RES (6)..(6): Gly or any amino acid from a heterologous signal peptide
  MOD_RES (7)..(7): Leu or any amino acid from a heterologous signal peptide
  MOD_RES (8)..(8): Ile or any amino acid from a heterologous signal peptide
  MOD_RES (9)..(9): Val or any amino acid from a heterologous signal peptide
  MOD_RES (10)..(11): Leu or any amino acid from a heterologous signal peptide
  MOD_RES (12)..(12): Gly or any amino acid from a heterologous signal peptide
  MOD_RES (13)..(13): Ser or any amino acid from a heterologous signal peptide
  MOD_RES (14)..(14): Trp or any amino acid from a heterologous signal peptide
  MOD_RES (15)..(15): Ser or any amino acid from a heterologous signal peptide
  MOD_RES (16)..(16): Leu or any amino acid from a heterologous signal peptide
  MOD_RES (17)..(17): Gly or any amino acid from a heterologous signal peptide
  MOD_RES (18)..(18): Asp or any amino acid from a heterologous signal peptide
  MOD_RES (19)..(19): Trp or any amino acid from a heterologous signal peptide
  MOD_RES (20)..(20): Gly or any amino acid from a heterologous signal peptide
  MOD_RES (21)..(21): Ala or any amino acid from a heterologous signal peptide
  MOD_RES (22)..(22): Glu or any amino acid from a heterologous signal peptide
  MOD_RES (23)..(23): Ala or any amino acid from a heterologous signal peptide
XXXXXXXXXXXXXXXXXXXXXXXCTCSPSHPQDAFCNSDIVIRAEVVGSKLVKEGPFGTLVYTIKQMKMYRGFTKMPHVQYIHTEASESLCGLKLEVNKYQYLLTGRVYDGKMYTGLCNFVERWDQLTLSQRKGLNYRYHLGCNCKIKSCYYLPCFVTSKNECLWTDMLSNFGYPGYQSKHYACIRQKGGYCSWYRGWAPPDKSIINATDP

SEQ ID NO: 6 - protein, 211 aa, Artificial Sequence
  Description of Artificial Sequence: Synthetic polypeptide
  MOD_RES (1)..(1): Met or any amino acid from a heterologous signal peptide
  MOD_RES (2)..(2): Thr or any amino acid from a heterologous signal peptide
  MOD_RES (3)..(3): Pro or any amino acid from a heterologous signal peptide
  MOD_RES (4)..(4): Trp or any amino acid from a heterologous signal peptide
  MOD_RES (5)..(5): Leu or any amino acid from a heterologous signal peptide
  MOD_RES (6)..(6): Gly or any amino acid from a heterologous signal peptide
  MOD_RES (7)..(7): Leu or any amino acid from a heterologous signal peptide
  MOD_RES (8)..(8): Ile or any amino acid from a heterologous signal peptide
  MOD_RES (9)..(9): Val or any amino acid from a heterologous signal peptide
  MOD_RES (10)..(11): Leu or any amino acid from a heterologous signal peptide
  MOD_RES (12)..(12): Gly or any amino acid from a heterologous signal peptide
  MOD_RES (13)..(13): Ser or any amino acid from a heterologous signal peptide
  MOD_RES (14)..(14): Trp or any amino acid from a heterologous signal peptide
  MOD_RES (15)..(15): Ser or any amino acid from a heterologous signal peptide
  MOD_RES (16)..(16): Leu or any amino acid from a heterologous signal peptide
  MOD_RES (17)..(17): Gly or any amino acid from a heterologous signal peptide
  MOD_RES (18)..(18): Asp or any amino acid from a heterologous signal peptide
  MOD_RES (19)..(19): Trp or any amino acid from a heterologous signal peptide
  MOD_RES (20)..(20): Gly or any amino acid from a heterologous signal peptide
  MOD_RES (21)..(21): Ala or any amino acid from a heterologous signal peptide
  MOD_RES (22)..(22): Glu or any amino acid from a heterologous signal peptide
  MOD_RES (23)..(23): Ala or any amino acid from a heterologous signal peptide
XXXXXXXXXXXXXXXXXXXXXXXCTCSPSHPQDAFCNSDIVIRAEVVGEKLVKEGPFGTLVYTIKQMKMYRGFTKMPHVQYIHTEASESLCGLKLEVNKYQYLLTGRVYDGKMYTGLCNFVERWDQLTLSQRKGLNYRYHLGCNCKIKSCYYLPCFVTSKNECLWTDMLSNFGYPGYQSKHYACIRQKGGYCSWYRGWAPPDKSIINATDP

SEQ ID NO: 7 - protein, 211 aa, Artificial Sequence
  Description of Artificial Sequence: Synthetic polypeptide
  MOD_RES (1)..(1): Met or any amino acid from a heterologous signal peptide
  MOD_RES (2)..(2): Thr or any amino acid from a heterologous signal peptide
  MOD_RES (3)..(3): Pro or any amino acid from a heterologous signal peptide
  MOD_RES (4)..(4): Trp or any amino acid from a heterologous signal peptide
  MOD_RES (5)..(5): Leu or any amino acid from a heterologous signal peptide
  MOD_RES (6)..(6): Gly or any amino acid from a heterologous signal peptide
  MOD_RES (7)..(7): Leu or any amino acid from a heterologous signal peptide
  MOD_RES (8)..(8): Ile or any amino acid from a heterologous signal peptide
  MOD_RES (9)..(9): Val or any amino acid from a heterologous signal peptide
  MOD_RES (10)..(11): Leu or any amino acid from a heterologous signal peptide
  MOD_RES (12)..(12): Gly or any amino acid from a heterologous signal peptide
  MOD_RES (13)..(13): Ser or any amino acid from a heterologous signal peptide
  MOD_RES (14)..(14): Trp or any amino acid from a heterologous signal peptide
  MOD_RES (15)..(15): Ser or any amino acid from a heterologous signal peptide
  MOD_RES (16)..(16): Leu or any amino acid from a heterologous signal peptide
  MOD_RES (17)..(17): Gly or any amino acid from a heterologous signal peptide
  MOD_RES (18)..(18): Asp or any amino acid from a heterologous signal peptide
  MOD_RES (19)..(19): Trp or any amino acid from a heterologous signal peptide
  MOD_RES (20)..(20): Gly or any amino acid from a heterologous signal peptide
  MOD_RES (21)..(21): Ala or any amino acid from a heterologous signal peptide
  MOD_RES (22)..(22): Glu or any amino acid from a heterologous signal peptide
  MOD_RES (23)..(23): Ala or any amino acid from a heterologous signal peptide
XXXXXXXXXXXXXXXXXXXXXXXCTCSPSHPQDAFCNSDIVIRAEVVGKKLVKEGPFGTLVYEIKQMKMYRGFTKMPHVQYIHTEASESLCGLKLEVNKYQYLLTGRVYDGKMYTGLCNFVERWDQLTLSQRKGLNYRYHLGCNCKIKSCYYLPCFVTSKNECLWTDMLSNFGYPGYQSKHYACIRQKGGYCSWYRGWAPPDKSIINATDP

SEQ ID NO: 8 - protein, 211 aa, Artificial Sequence
  Description of Artificial Sequence: Synthetic polypeptide
  MOD_RES (1)..(1): Met or any amino acid from a heterologous signal peptide
  MOD_RES (2)..(2): Thr or any amino acid from a heterologous signal peptide
  MOD_RES (3)..(3): Pro or any amino acid from a heterologous signal peptide
  MOD_RES (4)..(4): Trp or any amino acid from a heterologous signal peptide
  MOD_RES (5)..(5): Leu or any amino acid from a heterologous signal peptide
  MOD_RES (6)..(6): Gly or any amino acid from a heterologous signal peptide
  MOD_RES (7)..(7): Leu or any amino acid from a heterologous signal peptide
  MOD_RES (8)..(8): Ile or any amino acid from a heterologous signal peptide
  MOD_RES (9)..(9): Val or any amino acid from a heterologous signal peptide
  MOD_RES (10)..(11): Leu or any amino acid from a heterologous signal peptide
  MOD_RES (12)..(12): Gly or any amino acid from a heterologous signal peptide
  MOD_RES (13)..(13): Ser or any amino acid from a heterologous signal peptide
  MOD_RES (14)..(14): Trp or any amino acid from a heterologous signal peptide
  MOD_RES (15)..(15): Ser or any amino acid from a heterologous signal peptide
  MOD_RES (16)..(16): Leu or any amino acid from a heterologous signal peptide
  MOD_RES (17)..(17): Gly or any amino acid from a heterologous signal peptide
  MOD_RES (18)..(18): Asp or any amino acid from a heterologous signal peptide
  MOD_RES (19)..(19): Trp or any amino acid from a heterologous signal peptide
  MOD_RES (20)..(20): Gly or any amino acid from a heterologous signal peptide
  MOD_RES (21)..(21): Ala or any amino acid from a heterologous signal peptide
  MOD_RES (22)..(22): Glu or any amino acid from a heterologous signal peptide
  MOD_RES (23)..(23): Ala or any amino acid from a heterologous signal peptide
XXXXXXXXXXXXXXXXXXXXXXXCTCSPSHPQDAFCNSDIVIRAEVVGKKLVKEGPFGTLVYTIKQMKMYRGFTKMPHVEYIHTEASESLCGLKLEVNKYQYLLTGRVYDGKMYTGLCNFVERWDQLTLSQRKGLNYRYHLGCNCKIKSCYYLPCFVTSKNECLWTDMLSNFGYPGYQSKHYACIRQKGGYCSWYRGWAPPDKSIINATDP

SEQ ID NO: 9 - protein, 211 aa, Artificial Sequence
  Description of Artificial Sequence: Synthetic polypeptide
  MOD_RES (1)..(1): Met or any amino acid from a heterologous signal peptide
  MOD_RES (2)..(2): Thr or any amino acid from a heterologous signal peptide
  MOD_RES (3)..(3): Pro or any amino acid from a heterologous signal peptide
  MOD_RES (4)..(4): Trp or any amino acid from a heterologous signal peptide
  MOD_RES (5)..(5): Leu or any amino acid from a heterologous signal peptide
  MOD_RES (6)..(6): Gly or any amino acid from a heterologous signal peptide
  MOD_RES (7)..(7): Leu or any amino acid from a heterologous signal peptide
  MOD_RES (8)..(8): Ile or any amino acid from a heterologous signal peptide
  MOD_RES (9)..(9): Val or any amino acid from a heterologous signal peptide
  MOD_RES (10)..(11): Leu or any amino acid from a heterologous signal peptide
  MOD_RES (12)..(12): Gly or any amino acid from a heterologous signal peptide
  MOD_RES (13)..(13): Ser or any amino acid from a heterologous signal peptide
  MOD_RES (14)..(14): Trp or any amino acid from a heterologous signal peptide
  MOD_RES (15)..(15): Ser or any amino acid from a heterologous signal peptide
  MOD_RES (16)..(16): Leu or any amino acid from a heterologous signal peptide
  MOD_RES (17)..(17): Gly or any amino acid from a heterologous signal peptide
  MOD_RES (18)..(18): Asp or any amino acid from a heterologous signal peptide
  MOD_RES (19)..(19): Trp or any amino acid from a heterologous signal peptide
  MOD_RES (20)..(20): Gly or any amino acid from a heterologous signal peptide
  MOD_RES (21)..(21): Ala or any amino acid from a heterologous signal peptide
  MOD_RES (22)..(22): Glu or any amino acid from a heterologous signal peptide
  MOD_RES (23)..(23): Ala or any amino acid from a heterologous signal peptide
XXXXXXXXXXXXXXXXXXXXXXXCTCSPSHPQDAFCNSDIVIRAKVVGKKLVKEGPFGTLVYEIKQMKMYRGFTKMPEVQYIHTEASESLCGLKLEVNKYQYLLTGRVYDGKMYTGLCNFVERWDQLTLSQRKGLNYRYHLGCNCKIKSCYYLPCFVTSKNECLWTDMLSNFGYPGYQSKHYACIRQKGGYCSWYRGWAPPDKSIINATDP

SEQ ID NO: 10 - protein, 211 aa, Artificial Sequence
  Description of Artificial Sequence: Synthetic polypeptide
  MOD_RES (1)..(1): Met or any amino acid from a heterologous signal peptide
  MOD_RES (2)..(2): Thr or any amino acid from a heterologous signal peptide
  MOD_RES (3)..(3): Pro or any amino acid from a heterologous signal peptide
  MOD_RES (4)..(4): Trp or any amino acid from a heterologous signal peptide
  MOD_RES (5)..(5): Leu or any amino acid from a heterologous signal peptide
  MOD_RES (6)..(6): Gly or any amino acid from a heterologous signal peptide
  MOD_RES (7)..(7): Leu or any amino acid from a heterologous signal peptide
  MOD_RES (8)..(8): Ile or any amino acid from a heterologous signal peptide
  MOD_RES (9)..(9): Val or any amino acid from a heterologous signal peptide
  MOD_RES (10)..(11): Leu or any amino acid from a heterologous signal peptide
  MOD_RES (12)..(12): Gly or any amino acid from a heterologous signal peptide
  MOD_RES (13)..(13): Ser or any amino acid from a heterologous signal peptide
  MOD_RES (14)..(14): Trp or any amino acid from a heterologous signal peptide
  MOD_RES (15)..(15): Ser or any amino acid from a heterologous signal peptide
  MOD_RES (16)..(16): Leu or any amino acid from a heterologous signal peptide
  MOD_RES (17)..(17): Gly or any amino acid from a heterologous signal peptide
  MOD_RES (18)..(18): Asp or any amino acid from a heterologous signal peptide
  MOD_RES (19)..(19): Trp or any amino acid from a heterologous signal peptide
  MOD_RES (20)..(20): Gly or any amino acid from a heterologous signal peptide
  MOD_RES (21)..(21): Ala or any amino acid from a heterologous signal peptide
  MOD_RES (22)..(22): Glu or any amino acid from a heterologous signal peptide
  MOD_RES (23)..(23): Ala or any amino acid from a heterologous signal peptide
XXXXXXXXXXXXXXXXXXXXXXXCTCSPSHPQDAFCNSDIVIRAEVVGKKLVKEGPFGTLVYEIKQMKMYRGFTKMPEVQYIHTEASESLCGLKLEVNKYQYLLTGRVYDGKMYTGLCNFVERWDQLTLSQRKGLNYRYHLGCNCKIKSCYYLPCFVTSKNECLWTDMLSNFGYPGYQSKHYACIRQKGGYCSWYRGWAPPDKSIINATDP

SEQ ID NO: 11 - protein, 211 aa, Artificial Sequence
  Description of Artificial Sequence: Synthetic polypeptide
  MOD_RES (1)..(1): Met or any amino acid from a heterologous signal peptide
  MOD_RES (2)..(2): Thr or any amino acid from a heterologous signal peptide
  MOD_RES (3)..(3): Pro or any amino acid from a heterologous signal peptide
  MOD_RES (4)..(4): Trp or any amino acid from a heterologous signal peptide
  MOD_RES (5)..(5): Leu or any amino acid from a heterologous signal peptide
  MOD_RES (6)..(6): Gly or any amino acid from a heterologous signal peptide
  MOD_RES (7)..(7): Leu or any amino acid from a heterologous signal peptide
  MOD_RES (8)..(8): Ile or any amino acid from a heterologous signal peptide
  MOD_RES (9)..(9): Val or any amino acid from a heterologous signal peptide
  MOD_RES (10)..(11): Leu or any amino acid from a heterologous signal peptide
  MOD_RES (12)..(12): Gly or any amino acid from a heterologous signal peptide
  MOD_RES (13)..(13): Ser or any amino acid from a heterologous signal peptide
  MOD_RES (14)..(14): Trp or any amino acid from a heterologous signal peptide
  MOD_RES (15)..(15): Ser or any amino acid from a heterologous signal peptide
  MOD_RES (16)..(16): Leu or any amino acid from a heterologous signal peptide
  MOD_RES (17)..(17): Gly or any amino acid from a heterologous signal peptide
  MOD_RES (18)..(18): Asp or any amino acid from a heterologous signal peptide
  MOD_RES (19)..(19): Trp or any amino acid from a heterologous signal peptide
  MOD_RES (20)..(20): Gly or any amino acid from a heterologous signal peptide
  MOD_RES (21)..(21): Ala or any amino acid from a heterologous signal peptide
  MOD_RES (22)..(22): Glu or any amino acid from a heterologous signal peptide
  MOD_RES (23)..(23): Ala or any amino acid from a heterologous signal peptide
XXXXXXXXXXXXXXXXXXXXXXXCTCSPSHPQDAFCNSDIVIRAKVVGKKLVKEGPFGTLVYEIKQMKMYRGFTKMPEVEYIHTEASESLCGLKLEVNKYQYLLTGRVYDGKMYTGLCNFVERWDQLTLSQRKGLNYRYHLGCNCKIKSCYYLPCFVTSKNECLWTDMLSNFGYPGYQSKHYACIRQKGGYCSWYRGWAPPDKSIINATDP

SEQ ID NO: 12 - protein, 211 aa, Artificial Sequence
  Description of Artificial Sequence: Synthetic polypeptide
  MOD_RES (1)..(1): Met or any amino acid from a heterologous signal peptide
  MOD_RES (2)..(2): Thr or any amino acid from a heterologous signal peptide
  MOD_RES (3)..(3): Pro or any amino acid from a heterologous signal peptide
  MOD_RES (4)..(4): Trp or any amino acid from a heterologous signal peptide
  MOD_RES (5)..(5): Leu or any amino acid from a heterologous signal peptide
  MOD_RES (6)..(6): Gly or any amino acid from a heterologous signal peptide
  MOD_RES (7)..(7): Leu or any amino acid from a heterologous signal peptide
  MOD_RES (8)..(8): Ile or any amino acid from a heterologous signal peptide
  MOD_RES (9)..(9): Val or any amino acid from a heterologous signal peptide
  MOD_RES (10)..(11): Leu or any amino acid from a heterologous signal peptide
  MOD_RES (12)..(12): Gly or any amino acid from a heterologous signal peptide
  MOD_RES (13)..(13): Ser or any amino acid from a heterologous signal peptide
  MOD_RES (14)..(14): Trp or any amino acid from a heterologous signal peptide
  MOD_RES (15)..(15): Ser or any amino acid from a heterologous signal peptide
  MOD_RES (16)..(16): Leu or any amino acid from a heterologous signal peptide
  MOD_RES (17)..(17): Gly or any amino acid from a heterologous signal peptide
  MOD_RES (18)..(18): Asp or any amino acid from a heterologous signal peptide
  MOD_RES (19)..(19): Trp or any amino acid from a heterologous signal peptide
  MOD_RES (20)..(20): Gly or any amino acid from a heterologous signal peptide
  MOD_RES (21)..(21): Ala or any amino acid from a heterologous signal peptide
  MOD_RES (22)..(22): Glu or any amino acid from a heterologous signal peptide
  MOD_RES (23)..(23): Ala or any amino acid from a heterologous signal peptide
XXXXXXXXXXXXXXXXXXXXXXXCTCSPSHPQDAFCNSDIVIRAEVVGKKLVKEGPFGTLVYEIKQMKMYRGFTKMPEVEYIHTEASESLCGLKLEVNKYQYLLTGRVYDGKMYTGLCNFVERWDQLTLSQRKGLNYRYHLGCNCKIKSCYYLPCFVTSKNECLWTDMLSNFGYPGYQSKHYACIRQKGGYCSWYRGWAPPDKSIINATDP

SEQ ID NO: 13 - protein, 211 aa, Artificial Sequence
  Description of Artificial Sequence: Synthetic polypeptide
  MOD_RES (1)..(1): Met or any amino acid from a heterologous signal peptide
  MOD_RES (2)..(2): Thr or any amino acid from a heterologous signal peptide
  MOD_RES (3)..(3): Pro or any amino acid from a heterologous signal peptide
  MOD_RES (4)..(4): Trp or any amino acid from a heterologous signal peptide
  MOD_RES (5)..(5): Leu or any amino acid from a heterologous signal peptide
  MOD_RES (6)..(6): Gly or any amino acid from a heterologous signal peptide
  MOD_RES (7)..(7): Leu or any amino acid from a heterologous signal peptide
  MOD_RES (8)..(8): Ile or any amino acid from a heterologous signal peptide
  MOD_RES (9)..(9): Val or any amino acid from a heterologous signal peptide
  MOD_RES (10)..(11): Leu or any amino acid from a heterologous signal peptide
  MOD_RES (12)..(12): Gly or any amino acid from a heterologous signal peptide
  MOD_RES (13)..(13): Ser or any amino acid from a heterologous signal peptide
  MOD_RES (14)..(14): Trp or any amino acid from a heterologous signal peptide
  MOD_RES (15)..(15): Ser or any amino acid from a heterologous signal peptide
  MOD_RES (16)..(16): Leu or any amino acid from a heterologous signal peptide
  MOD_RES (17)..(17): Gly or any amino acid from a heterologous signal peptide
  MOD_RES (18)..(18): Asp or any amino acid from a heterologous signal peptide
  MOD_RES (19)..(19): Trp or any amino acid from a heterologous signal peptide
  MOD_RES (20)..(20): Gly or any amino acid from a heterologous signal peptide
  MOD_RES (21)..(21): Ala or any amino acid from a heterologous signal peptide
  MOD_RES (22)..(22): Glu or any amino acid from a heterologous signal peptide
  MOD_RES (23)..(23): Ala or any amino acid from a heterologous signal peptide
XXXXXXXXXXXXXXXXXXXXXXXCTCSPSHPQDAFCNSDIVIRAKVVGKKLVKEGPFGTLVYEIKQMKMYRGFEKMPEVQYIHTEASESLCGLKLEVNKYQYLLTGRVYDGKMYTGLCNFVERWDQLTLSQRKGLNYRYHLGCNCKIKSCYYLPCFVTSKNECLWTDMLSNFGYPGYQSKHYACIRQKGGYCSWYRGWAPPDKSIINATDP

SEQ ID NO: 14 - protein, 211 aa, Artificial Sequence
  Description of Artificial Sequence: Synthetic polypeptide
  MOD_RES (1)..(1): Met or any amino acid from a heterologous signal peptide
  MOD_RES (2)..(2): Thr or any amino acid from a heterologous signal peptide
  MOD_RES (3)..(3): Pro or any amino acid from a heterologous signal peptide
  MOD_RES (4)..(4): Trp or any amino acid from a heterologous signal peptide
  MOD_RES (5)..(5): Leu or any amino acid from a heterologous signal peptide
  MOD_RES (6)..(6): Gly or any amino acid from a heterologous signal peptide
  MOD_RES (7)..(7): Leu or any amino acid from a heterologous signal peptide
  MOD_RES (8)..(8): Ile or any amino acid from a heterologous signal peptide
  MOD_RES (9)..(9): Val or any amino acid from a heterologous signal peptide
  MOD_RES (10)..(11): Leu or any amino acid from a heterologous signal peptide
  MOD_RES (12)..(12): Gly or any amino acid from a heterologous signal peptide
  MOD_RES (13)..(13): Ser or any amino acid from a heterologous signal peptide
  MOD_RES (14)..(14): Trp or any amino acid from a heterologous signal peptide
  MOD_RES (15)..(15): Ser or any amino acid from a heterologous signal peptide
  MOD_RES (16)..(16): Leu or any amino acid from a heterologous signal peptide
  MOD_RES (17)..(17): Gly or any amino acid from a heterologous signal peptide
  MOD_RES (18)..(18): Asp or any amino acid from a heterologous signal peptide
  MOD_RES (19)..(19): Trp or any amino acid from a heterologous signal peptide
  MOD_RES (20)..(20): Gly or any amino acid from a heterologous signal peptide
  MOD_RES (21)..(21): Ala or any amino acid from a heterologous signal peptide
  MOD_RES (22)..(22): Glu or any amino acid from a heterologous signal peptide
  MOD_RES (23)..(23): Ala or any amino acid from a heterologous signal peptide
XXXXXXXXXXXXXXXXXXXXXXXCTCSPSHPQDAFCNSDIVIRAKVVGKKLVKEGPFGTLVYEIKQMKMYRGFEKMPDVQYIHTEASESLCGLKLEVNKYQYLLTGRVYDGKMYTGLCNFVERWDQLTLSQRKGLNYRYHLGCNCKIKSCYYLPCFVTSKNECLWTDMLSNFGYPGYQSKHYACIRQKGGYCSWYRGWAPPDKSIINATDP

SEQ ID NO: 15 - protein, 211 aa, Artificial Sequence
  Description of Artificial Sequence: Synthetic polypeptide
  MOD_RES (1)..(1): Met or any amino acid from a heterologous signal peptide
  MOD_RES (2)..(2): Thr or any amino acid from a heterologous signal peptide
  MOD_RES (3)..(3): Pro or any amino acid from a heterologous signal peptide
  MOD_RES (4)..(4): Trp or any amino acid from a heterologous signal peptide
  MOD_RES (5)..(5): Leu or any amino acid from a heterologous signal peptide
  MOD_RES (6)..(6): Gly or any amino acid from a heterologous signal peptide
  MOD_RES (7)..(7): Leu or any amino acid from a heterologous signal peptide
  MOD_RES (8)..(8): Ile or any amino acid from a heterologous signal peptide
  MOD_RES (9)..(9): Val or any amino acid from a heterologous signal peptide
  MOD_RES (10)..(11): Leu or any amino acid from a heterologous signal peptide
  MOD_RES (12)..(12): Gly or any amino acid from a heterologous signal peptide
  MOD_RES (13)..(13): Ser or any amino acid from a heterologous signal peptide
  MOD_RES (14)..(14): Trp or any amino acid from a heterologous signal peptide
  MOD_RES (15)..(15): Ser or any amino acid from a heterologous signal peptide
  MOD_RES (16)..(16): Leu or any amino acid from a heterologous signal peptide
  MOD_RES (17)..(17): Gly or any amino acid from a heterologous signal peptide
  MOD_RES (18)..(18): Asp or any amino acid from a heterologous signal peptide
  MOD_RES (19)..(19): Trp or any amino acid from a heterologous signal peptide
  MOD_RES (20)..(20): Gly or any amino acid from a heterologous signal peptide
  MOD_RES (21)..(21): Ala or any amino acid from a heterologous signal peptide
  MOD_RES (22)..(22): Glu or any amino acid from a heterologous signal peptide
  MOD_RES (23)..(23): Ala or any amino acid from a heterologous signal peptide
XXXXXXXXXXXXXXXXXXXXXXXCTCSPSHPQDAFCNSDIVIRAKVVGKKTVKEGPFGTLVYTIKQMKMYRGFEKMPDVQYIHTEASESLCGLKLEVNKYQYLLTGRVYDGKMYTGLCNFVERWDQLTLSQRKGLNYRYHLGCNCKIKSCYYLPCFVTSKNECLWTDMLSNFGYPGYQSKHYACIRQKGGYCSWYRGWAPPDKSIINATDP

SEQ ID NO: 16 - protein, 211 aa, Artificial Sequence
  Description of Artificial Sequence: Synthetic polypeptide
  MOD_RES (1)..(1): Met or any amino acid from a heterologous signal peptide
  MOD_RES (2)..(2): Thr or any amino acid from a heterologous signal peptide
  MOD_RES (3)..(3): Pro or any amino acid from a heterologous signal peptide
  MOD_RES (4)..(4): Trp or any amino acid from a heterologous signal peptide
  MOD_RES (5)..(5): Leu or any amino acid from a heterologous signal peptide
  MOD_RES (6)..(6): Gly or any amino acid from a heterologous signal peptide
  MOD_RES (7)..(7): Leu or any amino acid from a heterologous signal peptide
  MOD_RES (8)..(8): Ile or any amino acid from a heterologous signal peptide
  MOD_RES (9)..(9): Val or any amino acid from a heterologous signal peptide
  MOD_RES (10)..(11): Leu or any amino acid from a heterologous signal peptide
  MOD_RES (12)..(12): Gly or any amino acid from a heterologous signal peptide
  MOD_RES (13)..(13): Ser or any amino acid from a heterologous signal peptide
  MOD_RES (14)..(14): Trp or any amino acid from a heterologous signal peptide
  MOD_RES (15)..(15): Ser or any amino acid from a heterologous signal peptide
  MOD_RES (16)..(16): Leu or any amino acid from a heterologous signal peptide
  MOD_RES (17)..(17): Gly or any amino acid from a heterologous signal peptide
  MOD_RES (18)..(18): Asp or any amino acid from a heterologous signal peptide
  MOD_RES (19)..(19): Trp or any amino acid from a heterologous signal peptide
  MOD_RES (20)..(20): Gly or any amino acid from a heterologous signal peptide
  MOD_RES (21)..(21): Ala or any amino acid from a heterologous signal peptide
  MOD_RES (22)..(22): Glu or any amino acid from a heterologous signal peptide
  MOD_RES (23)..(23): Ala or any amino acid from a heterologous signal peptide
XXXXXXXXXXXXXXXXXXXXXXXCTCSPSHPQDAFCNSDIVIRAKVVGKKLVKEGPFGTLVYTIKQMKMYRGFEKMPEVEYIHTEASESLCGLKLEVNKYQYLLTGRVYDGKMYTGLCNFVERWDQLTLSQRKGLNYRYHLGCNCKIKSCYYLPCFVTSKNECLWTDMLSNFGYPGYQSKHYACIRQKGGYCSWYRGWAPPDKSIINATDP

SEQ ID NO: 17 - protein, 211 aa, Artificial Sequence
  Description of Artificial Sequence: Synthetic polypeptide
  MOD_RES (1)..(1): Met or any amino acid from a heterologous signal peptide
  MOD_RES (2)..(2): Thr or any amino acid from a heterologous signal peptide
  MOD_RES (3)..(3): Pro or any amino acid from a heterologous signal peptide
  MOD_RES (4)..(4): Trp or any amino acid from a heterologous signal peptide
  MOD_RES (5)..(5): Leu or any amino acid from a heterologous signal peptide
  MOD_RES (6)..(6): Gly or any amino acid from a heterologous signal peptide
  MOD_RES (7)..(7): Leu or any amino acid from a heterologous signal peptide
  MOD_RES (8)..(8): Ile or any amino acid from a heterologous signal peptide
  MOD_RES (9)..(9): Val or any amino acid from a heterologous signal peptide
  MOD_RES (10)..(11): Leu or any amino acid from a heterologous signal peptide
  MOD_RES (12)..(12): Gly or any amino acid from a heterologous signal peptide
  MOD_RES (13)..(13): Ser or any amino acid from a heterologous signal peptide
  MOD_RES (14)..(14): Trp or any amino acid from a heterologous signal peptide
  MOD_RES (15)..(15): Ser or any amino acid from a heterologous signal peptide
  MOD_RES (16)..(16): Leu or any amino acid from a heterologous signal peptide
  MOD_RES (17)..(17): Gly or any amino acid from a heterologous signal peptide
  MOD_RES (18)..(18): Asp or any amino acid from a heterologous signal peptide
  MOD_RES (19)..(19): Trp or any amino acid from a heterologous signal peptide
  MOD_RES (20)..(20): Gly or any amino acid from a heterologous signal peptide
  MOD_RES (21)..(21): Ala or any amino acid from a heterologous signal peptide
  MOD_RES (22)..(22): Glu or any amino acid from a heterologous signal peptide
  MOD_RES (23)..(23): Ala or any amino acid from a heterologous signal peptide
XXXXXXXXXXXXXXXXXXXXXXXCTCSPSHPQDAFCNSDIVIRAKVVGKKLVKEGPFGTLVYTIKQMKMYRGFEKMPDVEYIHTEASESLCGLKLEVNKYQYLLTGRVYDGKMYTGLCNFVERWDQLTLSQRKGLNYRYHLGCNCKIKSCYYLPCFVTSKNECLWTDMLSNFGYPGYQSKHYACIRQKGGYCSWYRGWAPPDKSIINATDP

SEQ ID NO: 18 - protein, 211 aa, Artificial Sequence
  Description of Artificial Sequence: Synthetic polypeptide
  MOD_RES (1)..(1): Met or any amino acid from a heterologous signal peptide
  MOD_RES (2)..(2): Thr or any amino acid from a heterologous signal peptide
  MOD_RES (3)..(3): Pro or any amino acid from a heterologous signal peptide
  MOD_RES (4)..(4): Trp or any amino acid from a heterologous signal peptide
  MOD_RES (5)..(5): Leu or any amino acid from a heterologous signal peptide
  MOD_RES (6)..(6): Gly or any amino acid from a heterologous signal peptide
  MOD_RES (7)..(7): Leu or any amino acid from a heterologous signal peptide
  MOD_RES (8)..(8): Ile or any amino acid from a heterologous signal peptide
  MOD_RES (9)..(9): Val or any amino acid from a heterologous signal peptide
  MOD_RES (10)..(11): Leu or any amino acid from a heterologous signal peptide
  MOD_RES (12)..(12): Gly or any amino acid from a heterologous signal peptide
  MOD_RES (13)..(13): Ser or any amino acid from a heterologous signal peptide
  MOD_RES (14)..(14): Trp or any amino acid from a heterologous signal peptide
  MOD_RES (15)..(15): Ser or any amino acid from a heterologous signal peptide
  MOD_RES (16)..(16): Leu or any amino acid from a heterologous signal peptide
  MOD_RES (17)..(17): Gly or any amino acid from a heterologous signal peptide
  MOD_RES (18)..(18): Asp or any amino acid from a heterologous signal peptide
  MOD_RES (19)..(19): Trp or any amino acid from a heterologous signal peptide
  MOD_RES (20)..(20): Gly or any amino acid from a heterologous signal peptide
  MOD_RES (21)..(21): Ala or any amino acid from a heterologous signal peptide
  MOD_RES (22)..(22): Glu or any amino acid from a heterologous signal peptide
  MOD_RES (23)..(23): Ala or any amino acid from a heterologous signal peptide
XXXXXXXXXXXXXXXXXXXXXXXCTCSPSHPQDAFCNSDIVIRANVTGKKLVKEGPFGTLVYEIKQMKMYRGFEKMPEVQYIHTEASESLCGLKLEVNKYQYLLTGRVYDGKMYTGLCNFVERWDQLTLSQRKGLNYRYHLGCNCKIKSCYYLPCFVTSKNECLWTDMLSNFGYPGYQSKHYACIRQKGGYCSWYRGWAPPDKSIINATDP

SEQ ID NO: 19 - protein, 211 aa, Artificial Sequence
  Description of Artificial Sequence: Synthetic polypeptide
  MOD_RES (1)..(1): Met or any amino acid from a heterologous signal peptide
  MOD_RES (2)..(2): Thr or any amino acid from a heterologous signal peptide
  MOD_RES (3)..(3): Pro or any amino acid from a heterologous signal peptide
  MOD_RES (4)..(4): Trp or any amino acid from a heterologous signal peptide
  MOD_RES (5)..(5): Leu or any amino acid from a heterologous signal peptide
  MOD_RES (6)..(6): Gly or any amino acid from a heterologous signal peptide
  MOD_RES (7)..(7): Leu or any amino acid from a heterologous signal peptide
  MOD_RES (8)..(8): Ile or any amino acid from a heterologous signal peptide
  MOD_RES (9)..(9): Val or any amino acid from a heterologous signal peptide
  MOD_RES (10)..(11): Leu or any amino acid from a heterologous signal peptide
  MOD_RES (12)..(12): Gly or any amino acid from a heterologous signal peptide
  MOD_RES (13)..(13): Ser or any amino acid from a heterologous signal peptide
  MOD_RES (14)..(14): Trp or any amino acid from a heterologous signal peptide
  MOD_RES (15)..(15): Ser or any amino acid from a heterologous signal peptide
  MOD_RES (16)..(16): Leu or any amino acid from a heterologous signal peptide
  MOD_RES (17)..(17): Gly or any amino acid from a heterologous signal peptide
  MOD_RES (18)..(18): Asp or any amino acid from a heterologous signal peptide
  MOD_RES (19)..(19): Trp or any amino acid from a heterologous signal peptide
  MOD_RES (20)..(20): Gly or any amino acid from a heterologous signal peptide
  MOD_RES (21)..(21): Ala or any amino acid from a heterologous signal peptide
  MOD_RES (22)..(22): Glu or any amino acid from a heterologous signal peptide
  MOD_RES (23)..(23): Ala or any amino acid from a heterologous signal peptide
XXXXXXXXXXXXXXXXXXXXXXXCTCSPSHPQDAFCNSDIVIRAKVVGNKTVKEGPFGTLVYEIKQMKMYRGFEKMPEVQYIHTEASESLCGLKLEVNKYQYLLTGRVYDGKMYTGLCNFVERWDQLTLSQRKGLNYRYHLGCNCKIKSCYYLPCFVTSKNECLWTDMLSNFGYPGYQSKHYACIRQKGGYCSWYRGWAPPDKSIINATDP

SEQ ID NO: 20 - protein, 211 aa, Artificial Sequence
  Description of Artificial Sequence: Synthetic polypeptide
  MOD_RES (1)..(1): Met or any amino acid from a heterologous signal peptide
  MOD_RES (2)..(2): Thr or any amino acid from a heterologous signal peptide
  MOD_RES (3)..(3): Pro or any amino acid from a heterologous signal peptide
  MOD_RES (4)..(4): Trp or any amino acid from a heterologous signal peptide
  MOD_RES (5)..(5): Leu or any amino acid from a heterologous signal peptide
  MOD_RES (6)..(6): Gly or any amino acid from a heterologous signal peptide
  MOD_RES (7)..(7): Leu or any amino acid from a heterologous signal peptide
  MOD_RES (8)..(8): Ile or any amino acid from a heterologous signal peptide
  MOD_RES (9)..(9): Val or any amino acid from a heterologous signal peptide
  MOD_RES (10)..(11): Leu or any amino acid from a heterologous signal peptide
  MOD_RES (12)..(12): Gly or any amino acid from a heterologous signal peptide
  MOD_RES (13)..(13): Ser or any amino acid from a heterologous signal peptide
  MOD_RES (14)..(14): Trp or any amino acid from a heterologous signal peptide
  MOD_RES (15)..(15): Ser or any amino acid from a heterologous signal peptide
  MOD_RES (16)..(16): Leu or any amino acid from a heterologous signal peptide
  MOD_RES (17)..(17): Gly or any amino acid from a heterologous signal peptide
  MOD_RES (18)..(18): Asp or any amino acid from a heterologous signal peptide
  MOD_RES (19)..(19): Trp or any amino acid from a heterologous signal peptide
  MOD_RES (20)..(20): Gly or any amino acid from a heterologous signal peptide
  MOD_RES (21)..(21): Ala or any amino acid from a heterologous signal peptide
  MOD_RES (22)..(22): Glu or any amino acid from a heterologous signal peptide
  MOD_RES (23)..(23): Ala or any amino acid from a heterologous signal peptide
XXXXXXXXXXXXXXXXXXXXXXXCTCSPSHPQDAFCNSDIVIRAEVVGNKTVKEGPFGTLVYEIKQMKMYRGFTKMPHVQYIHTEASESLCGLKLEVNKYQYLLTGRVYDGKMYTGLCNFVERWDQLTLSQRKGLNYRYHLGCNCKIKSCYYLPCFVTSKNECLWTDMLSNFGYPGYQSKHYACIRQKGGYCSWYRGWAPPDKSIINATDP

SEQ ID NO: 21 - protein, 211 aa, Artificial Sequence
  Description of Artificial Sequence: Synthetic polypeptide
  MOD_RES (1)..(1): Met or any amino acid from a heterologous signal peptide
  MOD_RES (2)..(2): Thr or any amino acid from a heterologous signal peptide
  MOD_RES (3)..(3): Pro or any amino acid from a heterologous signal peptide
  MOD_RES (4)..(4): Trp or any amino acid from a heterologous signal peptide
  MOD_RES (5)..(5): Leu or any amino acid from a heterologous signal peptide
  MOD_RES (6)..(6): Gly or any amino acid from a heterologous signal peptide
  MOD_RES (7)..(7): Leu or any amino acid from a heterologous signal peptide
  MOD_RES (8)..(8): Ile or any amino acid from a heterologous signal peptide
  MOD_RES (9)..(9): Val or any amino acid from a heterologous signal peptide
  MOD_RES (10)..(11): Leu or any amino acid from a heterologous signal peptide
  MOD_RES (12)..(12): Gly or any amino acid from a heterologous signal peptide
  MOD_RES (13)..(13): Ser or any amino acid from a heterologous signal peptide
  MOD_RES (14)..(14): Trp or any amino acid from a heterologous signal peptide
  MOD_RES (15)..(15): Ser or any amino acid from a heterologous signal peptide
  MOD_RES (16)..(16): Leu or any amino acid from a heterologous signal peptide
  MOD_RES (17)..(17): Gly or any amino acid from a heterologous signal peptide
  MOD_RES (18)..(18): Asp or any amino acid from a heterologous signal peptide
  MOD_RES (19)..(19): Trp or any amino acid from a heterologous signal peptide
  MOD_RES (20)..(20): Gly or any amino acid from a heterologous signal peptide
  MOD_RES (21)..(21): Ala or any amino acid from a heterologous signal peptide
  MOD_RES (22)..(22): Glu or any amino acid from a heterologous signal peptide
  MOD_RES (23)..(23): Ala or any amino acid from a heterologous signal peptide
XXXXXXXXXXXXXXXXXXXXXXXCTCSPSHPQDAFCNSDIVIRAKVVGNKTVKEGPFGTLVYTIKQMKMYRGFEKMPEVQYIHTEASESLCGLKLEVNKYQYLLTGRVYDGKMYTGLCNFVERWDQLTLSQRKGLNYRYHLGCNCKIKSCYYLPCFVTSKNECLWTDMLSNFGYPGYQSKHYACIRQKGGYCSWYRGWAPPDKSIINATDP

SEQ ID NO: 22 - protein, 211 aa, Artificial Sequence
  Description of Artificial Sequence: Synthetic polypeptide
  MOD_RES (1)..(1): Met or any amino acid from a heterologous signal peptide
  MOD_RES (2)..(2): Thr or any amino acid from a heterologous signal peptide
  MOD_RES (3)..(3): Pro or any amino acid from a heterologous signal peptide
  MOD_RES (4)..(4): Trp or any amino acid from a heterologous signal peptide
  MOD_RES (5)..(5): Leu or any amino acid from a heterologous signal peptide
  MOD_RES (6)..(6): Gly or any amino acid from a heterologous signal peptide
  MOD_RES (7)..(7): Leu or any amino acid from a heterologous signal peptide
  MOD_RES (8)..(8): Ile or any amino acid from a heterologous signal peptide
  MOD_RES (9)..(9): Val or any amino acid from a heterologous signal peptide
  MOD_RES (10)..(11): Leu or any amino acid from a heterologous signal peptide
  MOD_RES (12)..(12): Gly or any amino acid from a heterologous signal peptide
  MOD_RES (13)..(13): Ser or any amino acid from a heterologous signal peptide
  MOD_RES (14)..(14): Trp or any amino acid from a heterologous signal peptide
  MOD_RES (15)..(15): Ser or any amino acid from a heterologous signal peptide
  MOD_RES (16)..(16): Leu or any amino acid from a heterologous signal peptide
  MOD_RES (17)..(17): Gly or any amino acid from a heterologous signal peptide
  MOD_RES (18)..(18): Asp or any amino acid from a heterologous signal peptide
  MOD_RES (19)..(19): Trp or any amino acid from a heterologous signal peptide
  MOD_RES (20)..(20): Gly or any amino acid from a heterologous signal peptide
  MOD_RES (21)..(21): Ala or any amino acid from a heterologous signal peptide
  MOD_RES (22)..(22): Glu or any amino acid from a heterologous signal peptide
  MOD_RES (23)..(23): Ala or any amino acid from a heterologous signal peptide
XXXXXXXXXXXXXXXXXXXXXXXCTCSPSHPQDAFCNSDIVIRASVVGKKLVKEGPFGTLVYTIKQMKMYRGFTKMPHVQYIHTEASESLCGLKLEVNKYQYLLTGRVYDGKMYTGLCNFVERWDQLTLSQRKGLNYRYHLGCNCKIKSCYYLPCFVTSKNECLWTDMLSNFGYPGYQSKHYACIRQKGGYCSWYRGWAPPDKSIINATDP

SEQ ID NO: 23 - protein, 211 aa, Artificial Sequence
  Description of Artificial Sequence: Synthetic polypeptide
  MOD_RES (1)..(1): Met or any amino acid from a heterologous signal peptide
  MOD_RES (2)..(2): Thr or any amino acid from a heterologous signal peptide
  MOD_RES (3)..(3): Pro or any amino acid from a heterologous signal peptide
  MOD_RES (4)..(4): Trp or any amino acid from a heterologous signal peptide
  MOD_RES (5)..(5): Leu or any amino acid from a heterologous signal peptide
  MOD_RES (6)..(6): Gly or any amino acid from a heterologous signal peptide
  MOD_RES (7)..(7): Leu or any amino acid from a heterologous signal peptide
  MOD_RES (8)..(8): Ile or any amino acid from a heterologous signal peptide
  MOD_RES (9)..(9): Val or any amino acid from a heterologous signal peptide
  MOD_RES (10)..(11): Leu or any amino acid from a heterologous signal peptide
  MOD_RES (12)..(12): Gly or any amino acid from a heterologous signal peptide
  MOD_RES (13)..(13): Ser or any amino acid from a heterologous signal peptide
  MOD_RES (14)..(14): Trp or any amino acid from a heterologous signal peptide
  MOD_RES (15)..(15): Ser or any amino acid from a heterologous signal peptide
  MOD_RES (16)..(16): Leu or any amino acid from a heterologous signal peptide
  MOD_RES (17)..(17): Gly or any amino acid from a heterologous signal peptide
  MOD_RES (18)..(18): Asp or any amino acid from a heterologous signal peptide
  MOD_RES (19)..(19): Trp or any amino acid from a heterologous signal peptide
  MOD_RES (20)..(20): Gly or any amino acid from a heterologous signal peptide
  MOD_RES (21)..(21): Ala or any amino acid from a heterologous signal peptide
  MOD_RES (22)..(22): Glu or any amino acid from a heterologous signal peptide
  MOD_RES (23)..(23): Ala or any amino acid from a heterologous signal peptide
XXXXXXXXXXXXXXXXXXXXXXXCTCSPSHPQDAFCNSDIVIRASVVGKKLVKEGPNGTLVYTIKQMKMYRGFTKMPHVQYIHTEASESLCGLKLEVNKYQYLLTGRVYDGKMYTGLCNFVERWDQLTLSQRKGLNYRYHLGCNCKIKSCYYLPCFVTSKNECLWTDMLSNFGYPGYQSKHYACIRQKGGYCSWYRGWAPPDKSIINATDP

SEQ ID NO: 24 - protein, 211 aa, Artificial Sequence
  Description of Artificial Sequence: Synthetic polypeptide
  MOD_RES (1)..(1): Met or any amino acid from a heterologous signal peptide
  MOD_RES (2)..(2): Thr or any amino acid from a heterologous signal peptide
  MOD_RES (3)..(3): Pro or any amino acid from a heterologous signal peptide
  MOD_RES (4)..(4): Trp or any amino acid from a heterologous signal peptide
  MOD_RES (5)..(5): Leu or any amino acid from a heterologous signal peptide
  MOD_RES (6)..(6): Gly or any amino acid from a heterologous signal peptide
  MOD_RES (7)..(7): Leu or any amino acid from a heterologous signal peptide
  MOD_RES (8)..(8): Ile or any amino acid from a heterologous signal peptide
  MOD_RES (9)..(9): Val or any amino acid from a heterologous signal peptide
  MOD_RES (10)..(11): Leu or any amino acid from a heterologous signal peptide
  MOD_RES (12)..(12): Gly or any amino acid from a heterologous signal peptide
  MOD_RES (13)..(13): Ser or any amino acid from a heterologous signal peptide
  MOD_RES (14)..(14): Trp or any amino acid from a heterologous signal peptide
  MOD_RES (15)..(15): Ser or any amino acid from a heterologous signal peptide
  MOD_RES (16)..(16): Leu or any amino acid from a heterologous signal peptide
  MOD_RES (17)..(17): Gly or any amino acid from a heterologous signal peptide
  MOD_RES (18)..(18): Asp or any amino acid from a heterologous signal peptide
  MOD_RES (19)..(19): Trp or any amino acid from a heterologous signal peptide
  MOD_RES (20)..(20): Gly or any amino acid from a heterologous signal peptide
  MOD_RES (21)..(21): Ala or any amino acid from a heterologous signal peptide
  MOD_RES (22)..(22): Glu or any amino acid from a heterologous signal peptide
  MOD_RES (23)..(23): Ala or any amino acid from a heterologous signal peptide
XXXXXXXXXXXXXXXXXXXXXXXCTCSPSHPQDAFCNSDIVIRASVVGKKLVKEGPNGTLVYTIKQMKMYRGFTKMPHVQYIHTEASESLCGLKLEVNKYQYLLTGRVYDGKMYTGLCNFVERWDQLTLSQRSGLNYRYHLGCNCKIKSCYYLPCFVTSKNECLWTDMLSNFGYPGYQSKHYACIRQKGGYCSWYRGWAPPDKSIINATDP

SEQ ID NO: 25 - protein, 211 aa, Artificial Sequence; identical to SEQ ID NO: 17
  Description of Artificial Sequence: Synthetic polypeptide
  MOD_RES (1)..(1): Met or any amino acid from a heterologous signal peptide
  MOD_RES (2)..(2): Thr or any amino acid from a heterologous signal peptide
  MOD_RES (3)..(3): Pro or any amino acid from a heterologous signal peptide
  MOD_RES (4)..(4): Trp or any amino acid from a heterologous signal peptide
  MOD_RES (5)..(5): Leu or any amino acid from a heterologous signal peptide
  MOD_RES (6)..(6): Gly or any amino acid from a heterologous signal peptide
  MOD_RES (7)..(7): Leu or any amino acid from a heterologous signal peptide
  MOD_RES (8)..(8): Ile or any amino acid from a heterologous signal peptide
  MOD_RES (9)..(9): Val or any amino acid from a heterologous signal peptide
  MOD_RES (10)..(11): Leu or any amino acid from a heterologous signal peptide
  MOD_RES (12)..(12): Gly or any amino acid from a heterologous signal peptide
  MOD_RES (13)..(13): Ser or any amino acid from a heterologous signal peptide
  MOD_RES (14)..(14): Trp or any amino acid from a heterologous signal peptide
  MOD_RES (15)..(15): Ser or any amino acid from a heterologous signal peptide
  MOD_RES (16)..(16): Leu or any amino acid from a heterologous signal peptide
  MOD_RES (17)..(17): Gly or any amino acid from a heterologous signal peptide
  MOD_RES (18)..(18): Asp or any amino acid from a heterologous signal peptide
  MOD_RES (19)..(19): Trp or any amino acid from a heterologous signal peptide
  MOD_RES (20)..(20): Gly or any amino acid from a heterologous signal peptide
  MOD_RES (21)..(21): Ala or any amino acid from a heterologous signal peptide
  MOD_RES (22)..(22): Glu or any amino acid from a heterologous signal peptide
  MOD_RES (23)..(23): Ala or any amino acid from a heterologous signal peptide

SEQ ID NO: 26 - protein, 211 aa, Artificial Sequence
  Description of Artificial Sequence: Synthetic polypeptide
  MOD_RES (1)..(1): Met or any amino acid from a heterologous signal peptide
  MOD_RES (2)..(2): Thr or any amino acid from a heterologous signal peptide
  MOD_RES (3)..(3): Pro or any amino acid from a heterologous signal peptide
  MOD_RES (4)..(4): Trp or any amino acid from a heterologous signal peptide
  MOD_RES (5)..(5): Leu or any amino acid from a heterologous signal peptide
  MOD_RES (6)..(6): Gly or any amino acid from a heterologous signal peptide
  MOD_RES (7)..(7): Leu or any amino acid from a heterologous signal peptide
  MOD_RES (8)..(8): Ile or any amino acid from a heterologous signal peptide
  MOD_RES (9)..(9): Val or any amino acid from a heterologous signal peptide
  MOD_RES (10)..(11): Leu or any amino acid from a heterologous signal peptide
  MOD_RES (12)..(12): Gly or any amino acid from a heterologous signal peptide
  MOD_RES (13)..(13): Ser or any amino acid from a heterologous signal peptide
  MOD_RES (14)..(14): Trp or any amino acid from a heterologous signal peptide
  MOD_RES (15)..(15): Ser or any amino acid from a heterologous signal peptide
  MOD_RES (16)..(16): Leu or any amino acid from a heterologous signal peptide
  MOD_RES (17)..(17): Gly or any amino acid from a heterologous signal peptide
  MOD_RES (18)..(18): Asp or any amino acid from a heterologous signal peptide
  MOD_RES (19)..(19): Trp or any amino acid from a heterologous signal peptide
  MOD_RES (20)..(20): Gly or any amino acid from a heterologous signal peptide
  MOD_RES (21)..(21): Ala or any amino acid from a heterologous signal peptide
  MOD_RES (22)..(22): Glu or any amino acid from a heterologous signal peptide
  MOD_RES (23)..(23): Ala or any amino acid from a heterologous signal peptide
XXXXXXXXXXXXXXXXXXXXXXXCTCSPSHPQDAFCNSDIVIRANVTGKKLVKEGPFGTLVYTIKQMKMYRGFTKMPHVQYIHTEASESLCGLKLEVNKYQYLLTGRVYDGKMYTGLCNFVERWDQLTLSQRKGLNYRYHLGCNCKIKSCYYLPCFVTSKNECLWTDMLSNFGYPGYQSKHYACIRQKGGYCSWYRGWAPPDKSIINATDP

SEQ ID NO: 27 - protein, 211 aa, Artificial Sequence
  Description of Artificial Sequence: Synthetic polypeptide
  MOD_RES (1)..(1): Met or any amino acid from a heterologous signal peptide
  MOD_RES (2)..(2): Thr or any amino acid from a heterologous signal peptide
  MOD_RES (3)..(3): Pro or any amino acid from a heterologous signal peptide
  MOD_RES (4)..(4): Trp or any amino acid from a heterologous signal peptide
  MOD_RES (5)..(5): Leu or any amino acid from a heterologous signal peptide
  MOD_RES (6)..(6): Gly or any amino acid from a heterologous signal peptide
  MOD_RES (7)..(7): Leu or any amino acid from a heterologous signal peptide
  MOD_RES (8)..(8): Ile or any amino acid from a heterologous signal peptide
  MOD_RES (9)..(9): Val or any amino acid from a heterologous signal peptide
  MOD_RES (10)..(11): Leu or any amino acid from a heterologous signal peptide
  MOD_RES (12)..(12): Gly or any amino acid from a heterologous signal peptide
  MOD_RES (13)..(13): Ser or any amino acid from a heterologous signal peptide
  MOD_RES (14)..(14): Trp or any amino acid from a heterologous signal peptide
  MOD_RES (15)..(15): Ser or any amino acid from a heterologous signal peptide
  MOD_RES (16)..(16): Leu or any amino acid from a heterologous signal peptide
  MOD_RES (17)..(17): Gly or any amino acid from a heterologous signal peptide
  MOD_RES (18)..(18): Asp or any amino acid from a heterologous signal peptide
  MOD_RES (19)..(19): Trp or any amino acid from a heterologous signal peptide
  MOD_RES (20)..(20): Gly or any amino acid from a heterologous signal peptide
  MOD_RES (21)..(21): Ala or any amino acid from a heterologous signal peptide
  MOD_RES (22)..(22): Glu or any amino acid from a heterologous signal peptide
  MOD_RES (23)..(23): Ala or any amino acid from a heterologous signal peptide
XXXXXXXXXXXXXXXXXXXXXXXCTCSPSHPQDAFCNSDIVIRAKVVGNKTVKEGPFGTLVYTIKQMKMYRGFTKMPHVQYIHTEASESLCGLKLEVNKYQYLLTGRVYDGKMYTGLCNFVERWDQLTLSQRKGLNYRYHLGCNCKIKSCYYLPCFVTSKNECLWTDMLSNFGYPGYQSKHYACIRQKGGYCSWYRGWAPPDKSIINATDP

SEQ ID NO: 28 - protein, 211 aa, Artificial Sequence
  Description of Artificial Sequence: Synthetic polypeptide
  MOD_RES (1)..(1): Met or any amino acid from a heterologous signal peptide
  MOD_RES (2)..(2): Thr or any amino acid from a heterologous signal peptide
  MOD_RES (3)..(3): Pro or any amino acid from a heterologous signal peptide
  MOD_RES (4)..(4): Trp or any amino acid from a heterologous signal peptide
  MOD_RES (5)..(5): Leu or any amino acid from a heterologous signal peptide
  MOD_RES (6)..(6): Gly or any amino acid from a heterologous signal peptide
  MOD_RES (7)..(7): Leu or any amino acid from a heterologous signal peptide
  MOD_RES (8)..(8): Ile or any amino acid from a heterologous signal peptide
  MOD_RES (9)..(9): Val or any amino acid from a heterologous signal peptide
  MOD_RES (10)..(11): Leu or any amino acid from a heterologous signal peptide
  MOD_RES (12)..(12): Gly or any amino acid from a heterologous signal peptide
  MOD_RES (13)..(13): Ser or any amino acid from a heterologous signal peptide
  MOD_RES (14)..(14): Trp or any amino acid from a heterologous signal peptide
  MOD_RES (15)..(15): Ser or any amino acid from a heterologous signal peptide
  MOD_RES (16)..(16): Leu or any amino acid from a heterologous signal peptide
  MOD_RES (17)..(17): Gly or any amino acid from a heterologous signal peptide
  MOD_RES (18)..(18): Asp or any amino acid from a heterologous signal peptide
  MOD_RES (19)..(19): Trp or any amino acid from a heterologous signal peptide
  MOD_RES (20)..(20): Gly or any amino acid from a heterologous signal peptide
  MOD_RES (21)..(21): Ala or any amino acid from a heterologous signal peptide
  MOD_RES (22)..(22): Glu or any amino acid from a heterologous signal peptide
  MOD_RES (23)..(23): Ala or any amino acid from a heterologous signal peptide
XXXXXXXXXXXXXXXXXXXXXXXCTCSPSHPQDAFCNSDIVIRAKVVGSKLVKEGPNGTLVYTIKQMKMYRGFTKMPHVQYIHTEASESLCGLKLEVNKYQYLLTGRVYDGKMYTGLCNFVERWDQLTLSQRKGLNYRYHLGCNCKIKSCYYLPCFVTSKNECLWTDMLSNFGYPGYQSKHYACIRQKGGYCSWYRGWAPPDKSIINATDP

SEQ ID NO: 29 - protein, 211 aa, Artificial Sequence
  Description of Artificial Sequence: Synthetic polypeptide
  MOD_RES (1)..(1): Met or any amino acid from a heterologous signal peptide
  MOD_RES (2)..(2): Thr or any amino acid from a heterologous signal peptide
  MOD_RES (3)..(3): Pro or any amino acid from a heterologous signal peptide
  MOD_RES (4)..(4): Trp or any amino acid from a heterologous signal peptide
  MOD_RES (5)..(5): Leu or any amino acid from a heterologous signal peptide
  MOD_RES (6)..(6): Gly or any amino acid from a heterologous signal peptide
  MOD_RES (7)..(7): Leu or any amino acid from a heterologous signal peptide
  MOD_RES (8)..(8): Ile or any amino acid from a heterologous signal peptide
  MOD_RES (9)..(9): Val or any amino acid from a heterologous signal peptide
  MOD_RES (10)..(11): Leu or any amino acid from a heterologous signal peptide
  MOD_RES (12)..(12): Gly or any amino acid from a heterologous signal peptide
  MOD_RES (13)..(13): Ser or any amino acid from a heterologous signal peptide
  MOD_RES (14)..(14): Trp or any amino acid from a heterologous signal peptide
  MOD_RES (15)..(15): Ser or any amino acid from a heterologous signal peptide
  MOD_RES (16)..(16): Leu or any amino acid from a heterologous signal peptide
  MOD_RES (17)..(17): Gly or any amino acid from a heterologous signal peptide
  MOD_RES (18)..(18): Asp or any amino acid from a heterologous signal peptide
  MOD_RES (19)..(19): Trp or any amino acid from a heterologous signal peptide
  MOD_RES (20)..(20): Gly or any amino acid from a heterologous signal peptide
  MOD_RES (21)..(21): Ala or any amino acid from a heterologous signal peptide
  MOD_RES (22)..(22): Glu or any amino acid from a heterologous signal peptide
  MOD_RES (23)..(23): Ala or any amino acid from a heterologous signal peptide
XXXXXXXXXXXXXXXXXXXXXXXCTCSPSHPQDAFCNSDIVIRAKVVGSKLVKEGPNGTLVYTIKQMSMYRGFTKMPHVQYIHTEASESLCGLKLEVNKYQYLLTGRVYDGKMYTGLCNFVERWDQLTLSQRKGLNYRYHLGCNCKIKSCYYLPCFVTSKNECLWTDMLSNFGYPGYQSKHYACIRQKGGYCSWYRGWAPPDKSIINATDP

SEQ ID NO: 30 - protein, 211 aa, Artificial Sequence
  Description of Artificial Sequence: Synthetic polypeptide
  MOD_RES (1)..(1): Met or any amino acid from a heterologous signal peptide
  MOD_RES (2)..(2): Thr or any amino acid from a heterologous signal peptide
  MOD_RES (3)..(3): Pro or any amino acid from a heterologous signal peptide
  MOD_RES (4)..(4): Trp or any amino acid from a heterologous signal peptide
  MOD_RES (5)..(5): Leu or any amino acid from a heterologous signal peptide
  MOD_RES (6)..(6): Gly or any amino acid from a heterologous signal peptide
  MOD_RES (7)..(7): Leu or any amino acid from a heterologous signal peptide
  MOD_RES (8)..(8): Ile or any amino acid from a heterologous signal peptide
  MOD_RES (9)..(9): Val or any amino acid from a heterologous signal peptide
  MOD_RES (10)..(11): Leu or any amino acid from a heterologous signal peptide
  MOD_RES (12)..(12): Gly or any amino acid from a heterologous signal peptide
  MOD_RES (13)..(13): Ser or any amino acid from a heterologous signal peptide
  MOD_RES (14)..(14): Trp or any amino acid from a heterologous signal peptide
  MOD_RES (15)..(15): Ser or any amino acid from a heterologous signal peptide
  MOD_RES (16)..(16): Leu or any amino acid from a heterologous signal peptide
  MOD_RES (17)..(17): Gly or any amino acid from a heterologous signal peptide
  MOD_RES (18)..(18): Asp or any amino acid from a heterologous signal peptide
  MOD_RES (19)..(19): Trp or any amino acid from a heterologous signal peptide
  MOD_RES (20)..(20): Gly or any amino acid from a heterologous signal peptide
  MOD_RES (21)..(21): Ala or any amino acid from a heterologous signal peptide
  MOD_RES (22)..(22): Glu or any amino acid from a heterologous signal peptide
  MOD_RES (23)..(23): Ala or any amino acid from a heterologous signal peptide
XXXXXXXXXXXXXXXXXXXXXXXCTCSPSHPQDAFCNSDIVIRAKVVGKNLTKEGPFGTLVYTIKQMKMYRGFTKMPHVQYIHTEASESLCGLKLEVNKYQYLLTGRVYDGKMYTGLCNFVERWDQLTLSQRKGLNYRYHLGCNCKIKSCYYLPCFVTSKNECLWTDMLSNFGYPGYQSKHYACIRQKGGYCSWYRGWAPPDKSIINATDP

SEQ ID NO: 31 - protein, 211 aa, Artificial Sequence
  Description of Artificial Sequence: Synthetic polypeptide
  MOD_RES (1)..(1): Met or any amino acid from a heterologous signal peptide
  MOD_RES (2)..(2): Thr or any amino acid from a heterologous signal peptide
  MOD_RES (3)..(3): Pro or any amino acid from a heterologous signal peptide
  MOD_RES (4)..(4): Trp or any amino acid from a heterologous signal peptide
  MOD_RES (5)..(5): Leu or any amino acid from a heterologous signal peptide
  MOD_RES (6)..(6): Gly or any amino acid from a heterologous signal peptide
  MOD_RES (7)..(7): Leu or any amino acid from a heterologous signal peptide
  MOD_RES (8)..(8): Ile or any amino acid from a heterologous signal peptide
  MOD_RES (9)..(9): Val or any amino acid from a heterologous signal peptide
  MOD_RES (10)..(11): Leu or any amino acid from a heterologous signal peptide
  MOD_RES (12)..(12): Gly or any amino acid from a heterologous signal peptide
  MOD_RES (13)..(13): Ser or any amino acid from a heterologous signal peptide
  MOD_RES (14)..(14): Trp or any amino acid from a heterologous signal peptide
  MOD_RES (15)..(15): Ser or any amino acid from a heterologous signal peptide
  MOD_RES (16)..(16): Leu or any amino acid from a heterologous signal peptide
  MOD_RES (17)..(17): Gly or any amino acid from a heterologous signal peptide
  MOD_RES (18)..(18): Asp or any amino acid from a heterologous signal peptide
  MOD_RES (19)..(19): Trp or any amino acid from a heterologous signal peptide
  MOD_RES (20)..(20): Gly or any amino acid from a heterologous signal peptide
  MOD_RES (21)..(21): Ala or any amino acid from a heterologous signal peptide
  MOD_RES (22)..(22): Glu or any amino acid from a heterologous signal peptide
  MOD_RES (23)..(23): Ala or any amino acid from a heterologous signal peptide
XXXXXXXXXXXXXXXXXXXXXXXCTCSPSHPQDAFCNSDIVIRAKVVGKKLVKEGNFTTLVYTIKQMKMYRGFTKMPHVQYIHTEASESLCGLKLEVNKYQYLLTGRVYDGKMYTGLCNFVERWDQLTLSQRKGLNYRYHLGCNCKIKSCYYLPCFVTSKNECLWTDMLSNFGYPGYQSKHYACIRQKGGYCSWYRGWAPPDKSIINATDP

SEQ ID NO: 32 - protein, 211 aa, Artificial Sequence
  Description of Artificial Sequence: Synthetic polypeptide
  MOD_RES (1)..(1): Met or any amino acid from a heterologous signal peptide
  MOD_RES (2)..(2): Thr or any amino acid from a heterologous signal peptide
  MOD_RES (3)..(3): Pro or any amino acid from a heterologous signal peptide
  MOD_RES (4)..(4): Trp or any amino acid from a heterologous signal peptide
  MOD_RES (5)..(5): Leu or any amino acid from a heterologous signal peptide
  MOD_RES (6)..(6): Gly or any amino acid from a heterologous signal peptide
  MOD_RES (7)..(7): Leu or any amino acid from a heterologous signal peptide
  MOD_RES (8)..(8): Ile or any amino acid from a heterologous signal peptide
  MOD_RES (9)..(9): Val or any amino acid from a heterologous signal peptide
  MOD_RES (10)..(11): Leu or any amino acid from a heterologous signal peptide
  MOD_RES (12)..(12): Gly or any amino acid from a heterologous signal peptide
  MOD_RES (13)..(13): Ser or any amino acid from a heterologous signal peptide
  MOD_RES (14)..(14): Trp or any amino acid from a heterologous signal peptide
  MOD_RES (15)..(15): Ser or any amino acid from a heterologous signal peptide
  MOD_RES (16)..(16): Leu or any amino acid from a heterologous signal peptide
  MOD_RES (17)..(17): Gly or any amino acid from a heterologous signal peptide
  MOD_RES (18)..(18): Asp or any amino acid from a heterologous signal peptide
  MOD_RES (19)..(19): Trp or any amino acid from a heterologous signal peptide
  MOD_RES (20)..(20): Gly or any amino acid from a heterologous signal peptide
  MOD_RES (21)..(21): Ala or any amino acid from a heterologous signal peptide
  MOD_RES (22)..(22): Glu or any amino acid from a heterologous signal peptide
  MOD_RES (23)..(23): Ala or any amino acid from a heterologous signal peptide
XXXXXXXXXXXXXXXXXXXXXXXCTCSPSHPQDAFCNSDIVIRAKVVGKKLVKEGNFTTLVYNITQMKMYRGFTKMPHVQYIHTEASESLCGLKLEVNKYQYLLTGRVYDGKMYTGLCNFVERWDQLTLSQRKGLNYRYHLGCNCKIKSCYYLPCFVTSKNECLWTDMLSNFGYPGYQSKHYACIRQKGGYCSWYRGWAPPDKSIINATDP

SEQ ID NO: 33 - protein, 211 aa, Artificial Sequence
  Description of Artificial Sequence: Synthetic polypeptide
  MOD_RES (1)..(1): Met or any amino acid from a heterologous signal peptide
  MOD_RES (2)..(2): Thr or any amino acid from a heterologous signal peptide
  MOD_RES (3)..(3): Pro or any amino acid from a heterologous signal peptide
  MOD_RES (4)..(4): Trp or any amino acid from a heterologous signal peptide
  MOD_RES (5)..(5): Leu or any amino acid from a heterologous signal peptide
  MOD_RES (6)..(6): Gly or any amino acid from a heterologous signal peptide
  MOD_RES (7)..(7): Leu or any amino acid from a heterologous signal peptide
  MOD_RES (8)..(8): Ile or any amino acid from a heterologous signal peptide
  MOD_RES (9)..(9): Val or any amino acid from a heterologous signal peptide
  MOD_RES (10)..(11): Leu or any amino acid from a heterologous signal peptide
  MOD_RES (12)..(12): Gly or any amino acid from a heterologous signal peptide
  MOD_RES (13)..(13): Ser or any amino acid from a heterologous signal peptide
  MOD_RES (14)..(14): Trp or any amino acid from a heterologous signal peptide
  MOD_RES (15)..(15): Ser or any amino acid from a heterologous signal peptide
  MOD_RES (16)..(16): Leu or any amino acid from a heterologous signal peptide
  MOD_RES (17)..(17): Gly or any amino acid from a heterologous signal peptide
  MOD_RES (18)..(18): Asp or any amino acid from a heterologous signal peptide
  MOD_RES (19)..(19): Trp or any amino acid from a heterologous signal peptide
  MOD_RES (20)..(20): Gly or any amino acid from a heterologous signal peptide
  MOD_RES (21)..(21): Ala or any amino acid from a heterologous signal peptide
  MOD_RES (22)..(22): Glu or any amino acid from a heterologous signal peptide
  MOD_RES (23)..(23): Ala or any amino acid from a heterologous signal peptide
XXXXXXXXXXXXXXXXXXXXXXXCTCSPSHPQDAFCNSDIVIRAKVVGKKLVKEGPNGTLVYTIKQMKMYRGFTKMPHVQYIHTEASESLCGLKLEVNKYQYLLTGRVYDGKMYTGLCNFVERWDQLTLSQRKGLNYRYHLGCNCKIKSCYYLPCFVTSKNECLWTDMLSNFGYPGYQSKHYACIRQKGGYCSWYRGWAPPDKSIINATDP

SEQ ID NO: 34 - protein, 211 aa, Artificial Sequence
  Description of Artificial Sequence: Synthetic polypeptide
  MOD_RES (1)..(1): Met or any amino acid from a heterologous signal peptide
  MOD_RES (2)..(2): Thr or any amino acid from a heterologous signal peptide
  MOD_RES (3)..(3): Pro or any amino acid from a heterologous signal peptide
  MOD_RES (4)..(4): Trp or any amino acid from a heterologous signal peptide
  MOD_RES (5)..(5): Leu or any amino acid from a heterologous signal peptide
  MOD_RES (6)..(6): Gly or any amino acid from a heterologous signal peptide
  MOD_RES (7)..(7): Leu or any amino acid from a heterologous signal peptide
  MOD_RES (8)..(8): Ile or any amino acid from a heterologous signal peptide
  MOD_RES (9)..(9): Val or any amino acid from a heterologous signal peptide
  MOD_RES (10)..(11): Leu or any amino acid from a heterologous signal peptide
  MOD_RES (12)..(12): Gly or any amino acid from a heterologous signal peptide
  MOD_RES (13)..(13): Ser or any amino acid from a heterologous signal peptide
  MOD_RES (14)..(14): Trp or any amino acid from a heterologous signal peptide
  MOD_RES (15)..(15): Ser or any amino acid from a heterologous signal peptide
  MOD_RES (16)..(16): Leu or any amino acid from a heterologous signal peptide
  MOD_RES (17)..(17): Gly or any amino acid from a heterologous signal peptide
  MOD_RES (18)..(18): Asp or any amino acid from a heterologous signal peptide
  MOD_RES (19)..(19): Trp or any amino acid from a heterologous signal peptide
  MOD_RES (20)..(20): Gly or any amino acid from a heterologous signal peptide
  MOD_RES (21)..(21): Ala or any amino acid from a heterologous signal peptide
  MOD_RES (22)..(22): Glu or any amino acid from a heterologous signal peptide
  MOD_RES (23)..(23): Ala or any amino acid from a heterologous signal peptide
XXXXXXXXXXXXXXXXXXXXXXXCTCSPSHPQDAFCNSDIVIRAKVVGKKLVKEGPNGTLVYTIKQMSMYRGFTKMPHVQYIHTEASESLCGLKLEVNKYQYLLTGRVYDGKMYTGLCNFVERWDQLTLSQRKGLNYRYHLGCNCKIKSCYYLPCFVTSKNECLWTDMLSNFGYPGYQSKHYACIRQKGGYCSWYRGWAPPDKSIINATDP

SEQ ID NO: 35 - protein, 211 aa, Artificial Sequence
  Description of Artificial Sequence: Synthetic polypeptide
  MOD_RES (1)..(1): Met or any amino acid from a heterologous signal peptide
  MOD_RES (2)..(2): Thr or any amino acid from a heterologous signal peptide
  MOD_RES (3)..(3): Pro or any amino acid from a heterologous signal peptide
  MOD_RES (4)..(4): Trp or any amino acid from a heterologous signal peptide
  MOD_RES (5)..(5): Leu or any amino acid from a heterologous signal peptide
  MOD_RES (6)..(6): Gly or any amino acid from a heterologous signal peptide
  MOD_RES (7)..(7): Leu or any amino acid from a heterologous signal peptide
  MOD_RES (8)..(8): Ile or any amino acid from a heterologous signal peptide
  MOD_RES (9)..(9): Val or any amino acid from a heterologous signal peptide
  MOD_RES (10)..(11): Leu or any amino acid from a heterologous signal peptide
  MOD_RES (12)..(12): Gly or any amino acid from a heterologous signal peptide
  MOD_RES (13)..(13): Ser or any amino acid from a heterologous signal peptide
  MOD_RES (14)..(14): Trp or any amino acid from a heterologous signal peptide
  MOD_RES (15)..(15): Ser or any amino acid from a heterologous signal peptide
  MOD_RES (16)..(16): Leu or any amino acid from a heterologous signal peptide
  MOD_RES (17)..(17): Gly or any amino acid from a heterologous signal peptide
  MOD_RES (18)..(18): Asp or any amino acid from a heterologous signal peptide
  MOD_RES (19)..(19): Trp or any amino acid from a heterologous signal peptide
  MOD_RES (20)..(20): Gly or any amino acid from a heterologous signal peptide
  MOD_RES (21)..(21): Ala or any amino acid from a heterologous signal peptide
  MOD_RES (22)..(22): Glu or any amino acid from a heterologous signal peptide
  MOD_RES (23)..(23): Ala or any amino acid from a heterologous signal peptide
XXXXXXXXXXXXXXXXXXXXXXXCTCSPSHPQDAFCNSDIVIRAKVVGKKLVKEGPNGTLVYTIKQMKMYRGFTKMPHVQYIHTEASESLCGLKLEVNKYQYLLTGRVYDGKMYTGLCNFVERWDQLTLSQRSGLNYRYHLGCNCKIKSCYYLPCFVTSKNECLWTDMLSNFGYPGYQSKHYACIRQKGGYCSWYRGWAPPDKSIINATDP

SEQ ID NO: 36 - protein, 211 aa, Artificial Sequence
  Description of Artificial Sequence: Synthetic polypeptide
  MOD_RES (1)..(1): Met or any amino acid from a heterologous signal peptide
  MOD_RES (2)..(2): Thr or any amino acid from a heterologous signal peptide
  MOD_RES (3)..(3): Pro or any amino acid from a heterologous signal peptide
  MOD_RES (4)..(4): Trp or any amino acid from a heterologous signal peptide
  MOD_RES (5)..(5): Leu or any amino acid from a heterologous signal peptide
  MOD_RES (6)..(6): Gly or any amino acid from a heterologous signal peptide
  MOD_RES (7)..(7): Leu or any amino acid from a heterologous signal peptide
  MOD_RES (8)..(8): Ile or any amino acid from a heterologous signal peptide
  MOD_RES (9)..(9): Val or any amino acid from a heterologous signal peptide
  MOD_RES (10)..(11): Leu or any amino acid from a heterologous signal peptide
  MOD_RES (12)..(12): Gly or any amino acid from a heterologous signal peptide
  MOD_RES (13)..(13): Ser or any amino acid from a heterologous signal peptide
  MOD_RES (14)..(14): Trp or any amino acid from a heterologous signal peptide
  MOD_RES (15)..(15): Ser or any amino acid from a heterologous signal peptide
  MOD_RES (16)..(16): Leu or any amino acid from a heterologous signal peptide
  MOD_RES (17)..(17): Gly or any amino acid from a heterologous signal peptide
  MOD_RES (18)..(18): Asp or any amino acid from a heterologous signal peptide
  MOD_RES (19)..(19): Trp or any amino acid from a heterologous signal peptide
  MOD_RES (20)..(20): Gly or any amino acid from a heterologous signal peptide
  MOD_RES (21)..(21): Ala or any amino acid from a heterologous signal peptide
  MOD_RES (22)..(22): Glu or any amino acid from a heterologous signal peptide
  MOD_RES (23)..(23): Ala or any amino acid from a heterologous signal peptide
XXXXXXXXXXXXXXXXXXXXXXXCTCSPSHPQDAFCNSDIVIRAKVVGKKLVKEGPFGTLVYNITQMKMYRGFTKMPHVQYIHTEASESLCGLKLEVNKYQYLLTGRVYDGKMYTGLCNFVERWDQLTLSQRKGLNYRYHLGCNCKIKSCYYLPCFVTSKNECLWTDMLSNFGYPGYQSKHYACIRQKGGYCSWYRGWAPPDKSIINATDP

SEQ ID NO: 37 - protein, 211 aa, Artificial Sequence
  Description of Artificial Sequence: Synthetic polypeptide
  MOD_RES (1)..(1): Met or any amino acid from a heterologous signal peptide
  MOD_RES (2)..(2): Thr or any amino acid from a heterologous signal peptide
  MOD_RES (3)..(3): Pro or any amino acid from a heterologous signal peptide
  MOD_RES (4)..(4): Trp or any amino acid from a heterologous signal peptide
  MOD_RES (5)..(5): Leu or any amino acid from a heterologous signal peptide
  MOD_RES (6)..(6): Gly or any amino acid from a heterologous signal peptide
  MOD_RES (7)..(7): Leu or any amino acid from a heterologous signal peptide
  MOD_RES (8)..(8): Ile or any amino acid from a heterologous signal peptide
  MOD_RES (9)..(9): Val or any amino acid from a heterologous signal peptide
  MOD_RES (10)..(11): Leu or any amino acid from a heterologous signal peptide
  MOD_RES (12)..(12): Gly or any amino acid from a heterologous signal peptide
  MOD_RES (13)..(13): Ser or any amino acid from a heterologous signal peptide
  MOD_RES (14)..(14): Trp or any amino acid from a heterologous signal peptide
  MOD_RES (15)..(15): Ser or any amino acid from a heterologous signal peptide
  MOD_RES (16)..(16): Leu or any amino acid from a heterologous signal peptide
  MOD_RES (17)..(17): Gly or any amino acid from a heterologous signal peptide
  MOD_RES (18)..(18): Asp or any amino acid from a heterologous signal peptide
  MOD_RES (19)..(19): Trp or any amino acid from a heterologous signal peptide
  MOD_RES (20)..(20): Gly or any amino acid from a heterologous signal peptide
  MOD_RES (21)..(21): Ala or any amino acid from a heterologous signal peptide
  MOD_RES (22)..(22): Glu or any amino acid from a heterologous signal peptide
  MOD_RES (23)..(23): Ala or any amino acid from a heterologous signal peptide
XXXXXXXXXXXXXXXXXXXXXXXCTCSPSHPQDAFCNSDIVIRAKVVGKKLVKEGPFGTLVYTINQTKMYRGFTKMPHVQYIHTEASESLCGLKLEVNKYQYLLTGRVYDGKMYTGLCNFVERWDQLTLSQRKGLNYRYHLGCNCKIKSCYYLPCFVTSKNECLWTDMLSNFGYPGYQSKHYACIRQKGGYCSWYRGWAPPDKSIINATDP

SEQ ID NO: 38 - protein, 211 aa, Artificial Sequence
  Description of Artificial Sequence: Synthetic polypeptide
  MOD_RES (1)..(1): Met or any amino acid from a heterologous signal peptide
  MOD_RES (2)..(2): Thr or any amino acid from a heterologous signal peptide
  MOD_RES (3)..(3): Pro or any amino acid from a heterologous signal peptide
  MOD_RES (4)..(4): Trp or any amino acid from a heterologous signal peptide
  MOD_RES (5)..(5): Leu or any amino acid from a heterologous signal peptide
  MOD_RES (6)..(6): Gly or any amino acid from a heterologous signal peptide
  MOD_RES (7)..(7): Leu or any amino acid from a heterologous signal peptide
  MOD_RES (8)..(8): Ile or any amino acid from a heterologous signal peptide
  MOD_RES (9)..(9): Val or any amino acid from a heterologous signal peptide
  MOD_RES (10)..(11): Leu or any amino acid from a heterologous signal peptide
  MOD_RES (12)..(12): Gly or any amino acid from a heterologous signal peptide
  MOD_RES (13)..(13): Ser or any amino acid from a heterologous signal peptide
  MOD_RES (14)..(14): Trp or any amino acid from a heterologous signal peptide
  MOD_RES (15)..(15): Ser or any amino acid from a heterologous signal peptide
  MOD_RES (16)..(16): Leu or any amino acid from a heterologous signal peptide
  MOD_RES (17)..(17): Gly or any amino acid from a heterologous signal peptide
  MOD_RES (18)..(18): Asp or any amino acid from a heterologous signal peptide
  MOD_RES (19)..(19): Trp or any amino acid from a heterologous signal peptide
  MOD_RES (20)..(20): Gly or any amino acid from a heterologous signal peptide
  MOD_RES (21)..(21): Ala or any amino acid from a heterologous signal peptide
  MOD_RES (22)..(22): Glu or any amino acid from a heterologous signal peptide
  MOD_RES (23)..(23): Ala or any amino acid from a heterologous signal peptide
XXXXXXXXXXXXXXXXXXXXXXXCTCSPSHPQDAFCNSDIVIRAKVVGKKLVKEGPFGTLVYTIKQMKMYRGFTNMTHVQYIHTEASESLCGLKLEVNKYQYLLTGRVYDGKMYTGLCNFVERWDQLTLSQRKGLNYRYHLGCNCKIKSCYYLPCFVTSKNECLWTDMLSNFGYPGYQSKHYACIRQKGGYCSWYRGWAPPDKSIINATDP

SEQ ID NO: 39 - protein, 211 aa, Artificial Sequence
  Description of Artificial Sequence: Synthetic polypeptide
  MOD_RES (1)..(1): Met or any amino acid from a heterologous signal peptide
  MOD_RES (2)..(2): Thr or any amino acid from a heterologous signal peptide
  MOD_RES (3)..(3): Pro or any amino acid from a heterologous signal peptide
  MOD_RES (4)..(4): Trp or any amino acid from a heterologous signal peptide
  MOD_RES (5)..(5): Leu or any amino acid from a heterologous signal peptide
  MOD_RES (6)..(6): Gly or any amino acid from a heterologous signal peptide
  MOD_RES (7)..(7): Leu or any amino acid from a heterologous signal peptide
  MOD_RES (8)..(8): Ile or any amino acid from a heterologous signal peptide
  MOD_RES (9)..(9): Val or any amino acid from a heterologous signal peptide
  MOD_RES (10)..(11): Leu or any amino acid from a heterologous signal peptide
  MOD_RES (12)..(12): Gly or any amino acid from a heterologous signal peptide
  MOD_RES (13)..(13): Ser or any amino acid from a heterologous signal peptide
  MOD_RES (14)..(14): Trp or any amino acid from a heterologous signal peptide
  MOD_RES (15)..(15): Ser or any amino acid from a heterologous signal peptide
  MOD_RES (16)..(16): Leu or any amino acid from a heterologous signal peptide
  MOD_RES (17)..(17): Gly or any amino acid from a heterologous signal peptide
  MOD_RES (18)..(18): Asp or any amino acid from a heterologous signal peptide
  MOD_RES (19)..(19): Trp or any amino acid from a heterologous signal peptide
  MOD_RES (20)..(20): Gly or any amino acid from a heterologous signal peptide
  MOD_RES (21)..(21): Ala or any amino acid from a heterologous signal peptide
  MOD_RES (22)..(22): Glu or any amino acid from a heterologous signal peptide
  MOD_RES (23)..(23): Ala or any amino acid from a heterologous signal peptide
XXXXXXXXXXXXXXXXXXXXXXXCTCSPSHPQDAFCNSDIVIRAKVVGKKLVKEGPFGTLVYTIKQMKMYRGFTKMPNVTYIHTEASESLCGLKLEVNKYQYLLTGRVYDGKMYTGLCNFVERWDQLTLSQRKGLNYRYHLGCNCKIKSCYYLPCFVTSKNECLWTDMLSNFGYPGYQSKHYACIRQKGGYCSWYRGWAPPDKSIINATDP

SEQ ID NO: 40 - protein, 211 aa, Artificial Sequence
  Description of Artificial Sequence: Synthetic polypeptide
  MOD_RES (1)..(1): Met or any amino acid from a heterologous signal peptide
  MOD_RES (2)..(2): Thr or any amino acid from a heterologous signal peptide
  MOD_RES (3)..(3): Pro or any amino acid from a heterologous signal peptide
  MOD_RES (4)..(4): Trp or any amino acid from a heterologous signal peptide
  MOD_RES (5)..(5): Leu or any amino acid from a heterologous signal peptide
  MOD_RES (6)..(6): Gly or any amino acid from a heterologous signal peptide
  MOD_RES (7)..(7): Leu or any amino acid from a heterologous signal peptide
  MOD_RES (8)..(8): Ile or any amino acid from a heterologous signal peptide
  MOD_RES (9)..(9): Val or any amino acid from a heterologous signal peptide
  MOD_RES (10)..(11): Leu or any amino acid from a heterologous signal peptide
  MOD_RES (12)..(12): Gly or any amino acid from a heterologous signal peptide
  MOD_RES (13)..(13): Ser or any amino acid from a heterologous signal peptide
  MOD_RES (14)..(14): Trp or any amino acid from a heterologous signal peptide
  MOD_RES (15)..(15): Ser or any amino acid from a heterologous signal peptide
  MOD_RES (16)..(16): Leu or any amino acid from a heterologous signal peptide
  MOD_RES (17)..(17): Gly or any amino acid from a heterologous signal peptide
  MOD_RES (18)..(18): Asp or any amino acid from a heterologous signal peptide
  MOD_RES (19)..(19): Trp or any amino acid from a heterologous signal peptide
  MOD_RES (20)..(20): Gly or any amino acid from a heterologous signal peptide
  MOD_RES (21)..(21): Ala or any amino acid from a heterologous signal peptide
  MOD_RES (22)..(22): Glu or any amino acid from a heterologous signal peptide
  MOD_RES (23)..(23): Ala or any amino acid from a heterologous signal peptide
XXXXXXXXXXXXXXXXXXXXXXXCTCSPSHPQDAFCNSDIVIRAKVVGKKLVKEGPFGTLVYTIKQMKMYRGFTKMPHVQYIHTEASESLCGLNLTVNKYQYLLTGRVYDGKMYTGLCNFVERWDQLTLSQRKGLNYRYHLGCNCKIKSCYYLPCFVTSKNECLWTDMLSNFGYPGYQSKHYACIRQKGGYCSWYRGWAPPDKSIINATDP

SEQ ID NO: 41 - protein, 211 aa, Artificial Sequence
  Description of Artificial Sequence: Synthetic polypeptide
  MOD_RES (1)..(1): Met or any amino acid from a heterologous signal peptide
  MOD_RES (2)..(2): Thr or any amino acid from a heterologous signal peptide
  MOD_RES (3)..(3): Pro or any amino acid from a heterologous signal peptide
  MOD_RES (4)..(4): Trp or any amino acid from a heterologous signal peptide
  MOD_RES (5)..(5): Leu or any amino acid from a heterologous signal peptide
  MOD_RES (6)..(6): Gly or any amino acid from a heterologous signal peptide
  MOD_RES (7)..(7): Leu or any amino acid from a heterologous signal peptide
  MOD_RES (8)..(8): Ile or any amino acid from a heterologous signal peptide
  MOD_RES (9)..(9): Val or any amino acid from a heterologous signal peptide
  MOD_RES (10)..(11): Leu or any amino acid from a heterologous signal peptide
  MOD_RES (12)..(12): Gly or any amino acid from a heterologous signal peptide
  MOD_RES (13)..(13): Ser or any amino acid from a heterologous signal peptide
  MOD_RES (14)..(14): Trp or any amino acid from a heterologous signal peptide
  MOD_RES (15)..(15): Ser or any amino acid from a heterologous signal peptide
  MOD_RES (16)..(16): Leu or any amino acid from a heterologous signal peptide
  MOD_RES (17)..(17): Gly or any amino acid from a heterologous signal peptide
  MOD_RES (18)..(18): Asp or any amino acid from a heterologous signal peptide
  MOD_RES (19)..(19): Trp or any amino acid from a heterologous signal peptide
  MOD_RES (20)..(20): Gly or any amino acid from a heterologous signal peptide
  MOD_RES (21)..(21): Ala or any amino acid from a heterologous signal peptide
  MOD_RES (22)..(22): Glu or any amino acid from a heterologous signal peptide
  MOD_RES (23)..(23): Ala or any amino acid from a heterologous signal peptide
XXXXXXXXXXXXXXXXXXXXXXXCTCSPSHPQDAFCNSDIVIRAKVVGKKLVKEGPFGTLVYTIKQMKMYRGFTKMPHVQYIHTEASESLCGLKLNVTKYQYLLTGRVYDGKMYTGLCNFVERWDQLTLSQRKGLNYRYHLGCNCKIKSCYYLPCFVTSKNECLWTDMLSNFGYPGYQSKHYACIRQKGGYCSWYRGWAPPDKSIINATDP

SEQ ID NO: 42 - protein, 211 aa, Artificial Sequence
  Description of Artificial Sequence: Synthetic polypeptide
  MOD_RES (1)..(1): Met or any amino acid from a heterologous signal peptide
  MOD_RES (2)..(2): Thr or any amino acid from a heterologous signal peptide
  MOD_RES (3)..(3): Pro or any amino acid from a heterologous signal peptide
  MOD_RES (4)..(4): Trp or any amino acid from a heterologous signal peptide
  MOD_RES (5)..(5): Leu or any amino acid from a heterologous signal peptide
  MOD_RES (6)..(6): Gly or any amino acid from a heterologous signal peptide
  MOD_RES (7)..(7): Leu or any amino acid from a heterologous signal peptide
  MOD_RES (8)..(8): Ile or any amino acid from a heterologous signal peptide
  MOD_RES (9)..(9): Val or any amino acid from a heterologous signal peptide
  MOD_RES (10)..(11): Leu or any amino acid from a heterologous signal peptide
  MOD_RES (12)..(12): Gly or any amino acid from a heterologous signal peptide
  MOD_RES (13)..(13): Ser or any amino acid from a heterologous signal peptide
  MOD_RES (14)..(14): Trp or any amino acid from a heterologous signal peptide
  MOD_RES (15)..(15): Ser or any amino acid from a heterologous signal peptide
  MOD_RES (16)..(16): Leu or any amino acid from a heterologous signal peptide
  MOD_RES (17)..(17): Gly or any amino acid from a heterologous signal peptide
  MOD_RES (18)..(18): Asp or any amino acid from a heterologous signal peptide
  MOD_RES (19)..(19): Trp or any amino acid from a heterologous signal peptide
  MOD_RES (20)..(20): Gly or any amino acid from a heterologous signal peptide
  MOD_RES (21)..(21): Ala or any amino acid from a heterologous signal peptide
  MOD_RES (22)..(22): Glu or any amino acid from a heterologous signal peptide
  MOD_RES (23)..(23): Ala or any amino acid from a heterologous signal peptide
XXXXXXXXXXXXXXXXXXXXXXXCTCSPSHPQDAFCNSDIVIRAKVVGKKLVKEGPFGTLVYTIKQMKMYRGFTKMPHVQYIHTEASESLCGLKLENNTYQYLLTGRVYDGKMYTGLCNFVERWDQLTLSQRKGLNYRYHLGCNCKIKSCYYLPCFVTSKNECLWTDMLSNFGYPGYQSKHYACIRQKGGYCSWYRGWAPPDKSIINATDP

SEQ ID NO: 43 - protein, 211 aa, Artificial Sequence
  Description of Artificial Sequence: Synthetic polypeptide
  MOD_RES (1)..(1): Met or any amino acid from a heterologous signal peptide
  MOD_RES (2)..(2): Thr or any amino acid from a heterologous signal peptide
  MOD_RES (3)..(3): Pro or any amino acid from a heterologous signal peptide
  MOD_RES (4)..(4): Trp or any amino acid from a heterologous signal peptide
  MOD_RES (5)..(5): Leu or any amino acid from a heterologous signal peptide
  MOD_RES (6)..(6): Gly or any amino acid from a heterologous signal peptide
  MOD_RES (7)..(7): Leu or any amino acid from a heterologous signal peptide
  MOD_RES (8)..(8): Ile or any amino acid from a heterologous signal peptide
  MOD_RES (9)..(9): Val or any amino acid from a heterologous signal peptide
  MOD_RES (10)..(11): Leu or any amino acid from a heterologous signal peptide
  MOD_RES (12)..(12): Gly or any amino acid from a heterologous signal peptide
  MOD_RES (13)..(13): Ser or any amino acid from a heterologous signal peptide
  MOD_RES (14)..(14): Trp or any amino acid from a heterologous signal peptide
  MOD_RES (15)..(15): Ser or any amino acid from a heterologous signal peptide
  MOD_RES (16)..(16): Leu or any amino acid from a heterologous signal peptide
  MOD_RES (17)..(17): Gly or any amino acid from a heterologous signal peptide
  MOD_RES (18)..(18): Asp or any amino acid from a heterologous signal peptide
  MOD_RES (19)..(19): Trp or any amino acid from a heterologous signal peptide
  MOD_RES (20)..(20): Gly or any amino acid from a heterologous signal peptide
  MOD_RES (21)..(21): Ala or any amino acid from a heterologous signal peptide
  MOD_RES (22)..(22): Glu or any amino acid from a heterologous signal peptide
  MOD_RES (23)..(23): Ala or any amino acid from a heterologous signal peptide
XXXXXXXXXXXXXXXXXXXXXXXCTCSPSHPQDAFCNSDIVIRAKVVGKKLVKEGPFGTLVYTIKQMKMYRGFTKMPHVQYIHTEASESLCGLKLEVNKYQYLLTGRVYNGTMYTGLCNFVERWDQLTLSQRKGLNYRYHLGCNCKIKSCYYLPCFVTSKNECLWTDMLSNFGYPGYQSKHYACIRQKGGYCSWYRGWAPPDKSIINATDP

SEQ ID NO: 44 - protein, 211 aa, Artificial Sequence
  Description of Artificial Sequence: Synthetic polypeptide
  MOD_RES (1)..(1): Met or any amino acid from a heterologous signal peptide
  MOD_RES (2)..(2): Thr or any amino acid from a heterologous signal peptide
  MOD_RES (3)..(3): Pro or any amino acid from a heterologous signal peptide
  MOD_RES (4)..(4): Trp or any amino acid from a heterologous signal peptide
  MOD_RES (5)..(5): Leu or any amino acid from a heterologous signal peptide
  MOD_RES (6)..(6): Gly or any amino acid from a heterologous signal peptide
  MOD_RES (7)..(7): Leu or any amino acid from a heterologous signal peptide
  MOD_RES (8)..(8): Ile or any amino acid from a heterologous signal peptide
  MOD_RES (9)..(9): Val or any amino acid from a heterologous signal peptide
  MOD_RES (10)..(11): Leu or any amino acid from a heterologous signal peptide
  MOD_RES (12)..(12): Gly or any amino acid from a heterologous signal peptide
  MOD_RES (13)..(13): Ser or any amino acid from a heterologous signal peptide
  MOD_RES (14)..(14): Trp or any amino acid from a heterologous signal peptide
  MOD_RES (15)..(15): Ser or any amino acid from a heterologous signal peptide
  MOD_RES (16)..(16): Leu or any amino acid from a heterologous signal peptide
  MOD_RES (17)..(17): Gly or any amino acid from a heterologous signal peptide
  MOD_RES (18)..(18): Asp or any amino acid from a heterologous signal peptide
  MOD_RES (19)..(19): Trp or any amino acid from a heterologous signal peptide
  MOD_RES (20)..(20): Gly or any amino acid from a heterologous signal peptide
  MOD_RES (21)..(21): Ala or any amino acid from a heterologous signal peptide
  MOD_RES (22)..(22): Glu or any amino acid from a heterologous signal peptide
  MOD_RES (23)..(23): Ala or any amino acid from a heterologous signal peptide
XXXXXXXXXXXXXXXXXXXXXXXCTCSPSHPQDAFCNSDIVIRAKVVGKKLVKEGPFGTLVYTIKQMKMYRGFTKMPHVQYIHTEASESLCGLKLEVNKYQYLLTGRVYDGKMYTGLCNFVERWDNLTLSQRKGLNYRYHLGCNCKIKSCYYLPCFVTSKNECLWTDMLSNFGYPGYQSKHYACIRQKGGYCSWYRGWAPPDKSIINATDP

SEQ ID NO: 45 - protein, 211 aa, Artificial Sequence
  Description of Artificial Sequence: Synthetic polypeptide
  MOD_RES (1)..(1): Met or any amino acid from a heterologous signal peptide
  MOD_RES (2)..(2): Thr or any amino acid from a heterologous signal peptide
  MOD_RES (3)..(3): Pro or any amino acid from a heterologous signal peptide
  MOD_RES (4)..(4): Trp or any amino acid from a heterologous signal peptide
  MOD_RES (5)..(5): Leu or any amino acid from a heterologous signal peptide
  MOD_RES (6)..(6): Gly or any amino acid from a heterologous signal peptide
  MOD_RES (7)..(7): Leu or any amino acid from a heterologous signal peptide
  MOD_RES (8)..(8): Ile or any amino acid from a heterologous signal peptide
  MOD_RES (9)..(9): Val or any amino acid from a heterologous signal peptide
  MOD_RES (10)..(11): Leu or any amino acid from a heterologous signal peptide
  MOD_RES (12)..(12): Gly or any amino acid from a heterologous signal peptide
  MOD_RES (13)..(13): Ser or any amino acid from a heterologous signal peptide
  MOD_RES (14)..(14): Trp or any amino acid from a heterologous signal peptide
  MOD_RES (15)..(15): Ser or any amino acid from a heterologous signal peptide
  MOD_RES (16)..(16): Leu or any amino acid from a heterologous signal peptide
  MOD_RES (17)..(17): Gly or any amino acid from a heterologous signal peptide
  MOD_RES (18)..(18): Asp or any amino acid from a heterologous signal peptide
  MOD_RES (19)..(19): Trp or any amino acid from a heterologous signal peptide
  MOD_RES (20)..(20): Gly or any amino acid from a heterologous signal peptide
  MOD_RES (21)..(21): Ala or any amino acid from a heterologous signal peptide
  MOD_RES (22)..(22): Glu or any amino acid from a heterologous signal peptide
  MOD_RES (23)..(23): Ala or any amino acid from a heterologous signal peptide
XXXXXXXXXXXXXXXXXXXXXXXCTCSPSHPQDAFCNSDIVIRAKVVGKKLVKEGPFGTLVYTIKQMKMYRGFTKMPHVQYIHTEASESLCGLKLEVNKYQYLLTGRVYDGKMYTGLCNFVERWDQLTLSQRKGLNYTYHLGCNCKIKSCYYLPCFVTSKNECLWTDMLSNFGYPGYQSKHYACIRQKGGYCSWYRGWAPPDKSIINATDP

SEQ ID NO: 46 - protein, 211 aa, Artificial Sequence
  Description of Artificial Sequence: Synthetic polypeptide
  MOD_RES (1)..(1): Met or any amino acid from a heterologous signal peptide
  MOD_RES (2)..(2): Thr or any amino acid from a heterologous signal peptide
  MOD_RES (3)..(3): Pro or any amino acid from a heterologous signal peptide
  MOD_RES (4)..(4): Trp or any amino acid from a heterologous signal peptide
  MOD_RES (5)..(5): Leu or any amino acid from a heterologous signal peptide
  MOD_RES (6)..(6): Gly or any amino acid from a heterologous signal peptide
  MOD_RES (7)..(7): Leu or any amino acid from a heterologous signal peptide
  MOD_RES (8)..(8): Ile or any amino acid from a heterologous signal peptide
  MOD_RES (9)..(9): Val or any amino acid from a heterologous signal peptide
  MOD_RES (10)..(11): Leu or any amino acid from a heterologous signal peptide
  MOD_RES (12)..(12): Gly or any amino acid from a heterologous signal peptide
  MOD_RES (13)..(13): Ser or any amino acid from a heterologous signal peptide
  MOD_RES (14)..(14): Trp or any amino acid from a heterologous signal peptide
  MOD_RES (15)..(15): Ser or any amino acid from a heterologous signal peptide
  MOD_RES (16)..(16): Leu or any amino acid from a heterologous signal peptide
  MOD_RES (17)..(17): Gly or any amino acid from a heterologous signal peptide
  MOD_RES (18)..(18): Asp or any amino acid from a heterologous signal peptide
  MOD_RES (19)..(19): Trp or any amino acid from a heterologous signal peptide
  MOD_RES (20)..(20): Gly or any amino acid from a heterologous signal peptide
  MOD_RES (21)..(21): Ala or any amino acid from a heterologous signal peptide
  MOD_RES (22)..(22): Glu or any amino acid from a heterologous signal peptide
  MOD_RES (23)..(23): Ala or any amino acid from a heterologous signal peptide
XXXXXXXXXXXXXXXXXXXXXXXCTCSPSHPQDAFCNSDIVIRAKVVGKKLVKEGPFGTLVYTIKQMKMYRGFTKMPHVQYIHTEASESLCGLKLEVNKYQYLLTGRVYDGKMYTGLCNFVERWDQLTLSQRKGLNYNYTLGCNCKIKSCYYLPCFVTSKNECLWTDMLSNFGYPGYQSKHYACIRQKGGYCSWYRGWAPPDKSIINATDP

SEQ ID NO: 47 - protein, 211 aa, Artificial Sequence
  Description of Artificial Sequence: Synthetic polypeptide
  MOD_RES (1)..(1): Met or any amino acid from a heterologous signal peptide
  MOD_RES (2)..(2): Thr or any amino acid from a heterologous signal peptide
  MOD_RES (3)..(3): Pro or any amino acid from a heterologous signal peptide
  MOD_RES (4)..(4): Trp or any amino acid from a heterologous signal peptide
  MOD_RES (5)..(5): Leu or any amino acid from a heterologous signal peptide
  MOD_RES (6)..(6): Gly or any amino acid from a heterologous signal peptide
  MOD_RES (7)..(7): Leu or any amino acid from a heterologous signal peptide
  MOD_RES (8)..(8): Ile or any amino acid from a heterologous signal peptide
  MOD_RES (9)..(9): Val or any amino acid from a heterologous signal peptide
  MOD_RES (10)..(11): Leu or any amino acid from a heterologous signal peptide
  MOD_RES (12)..(12): Gly or any amino acid from a heterologous signal peptide
  MOD_RES (13)..(13): Ser or any amino acid from a heterologous signal peptide
  MOD_RES (14)..(14): Trp or any amino acid from a heterologous signal peptide
  MOD_RES (15)..(15): Ser or any amino acid from a heterologous signal peptide
  MOD_RES (16)..(16): Leu or any amino acid from a heterologous signal peptide
  MOD_RES (17)..(17): Gly or any amino acid from a heterologous signal peptide
  MOD_RES (18)..(18): Asp or any amino acid from a heterologous signal peptide
  MOD_RES (19)..(19): Trp or any amino acid from a heterologous signal peptide
  MOD_RES (20)..(20): Gly or any amino acid from a heterologous signal peptide
  MOD_RES (21)..(21): Ala or any amino acid from a heterologous signal peptide
  MOD_RES (22)..(22): Glu or any amino acid from a heterologous signal peptide
  MOD_RES (23)..(23): Ala or any amino acid from a heterologous signal peptide
XXXXXXXXXXXXXXXXXXXXXXXCTCSPSHPQDAFCNSDIVIRAKVVGKKLVKEGPFGTLVYTIKQMKMYRGFTKMPHVQYIHTEASESLCGLKLEVNKYQYLLTGRVYDGKMYTGLCNFVERWDQLTLSQRKGLNYRYHLGCNCKIKSCYYLPCFVNSTNECLWTDMLSNFGYPGYQSKHYACIRQKGGYCSWYRGWAPPDKSIINATDP

SEQ ID NO: 48 - protein, 211 aa, Artificial Sequence
  Description of Artificial Sequence: Synthetic polypeptide
  MOD_RES (1)..(1): Met or any amino acid from a heterologous signal peptide
  MOD_RES (2)..(2): Thr or any amino acid from a heterologous signal peptide
  MOD_RES (3)..(3): Pro or any amino acid from a heterologous signal peptide
  MOD_RES (4)..(4): Trp or any amino acid from a heterologous signal peptide
  MOD_RES (5)..(5): Leu or any amino acid from a heterologous signal peptide
  MOD_RES (6)..(6): Gly or any amino acid from a heterologous signal peptide
  MOD_RES (7)..(7): Leu or any amino acid from a heterologous signal peptide
  MOD_RES (8)..(8): Ile or any amino acid from a heterologous signal peptide
  MOD_RES (9)..(9): Val or any amino acid from a heterologous signal peptide
  MOD_RES (10)..(11): Leu or any amino acid from a heterologous signal peptide
  MOD_RES (12)..(12): Gly or any amino acid from a heterologous signal peptide
  MOD_RES (13)..(13): Ser or any amino acid from a heterologous signal peptide
  MOD_RES (14)..(14): Trp or any amino acid from a heterologous signal peptide
  MOD_RES (15)..(15): Ser or any amino acid from a heterologous signal peptide
  MOD_RES (16)..(16): Leu or any amino acid from a heterologous signal peptide
  MOD_RES (17)..(17): Gly or any amino acid from a heterologous signal peptide
  MOD_RES (18)..(18): Asp or any amino acid from a heterologous signal peptide
  MOD_RES (19)..(19): Trp or any amino acid from a heterologous signal peptide
  MOD_RES (20)..(20): Gly or any amino acid from a heterologous signal peptide
  MOD_RES (21)..(21): Ala or any amino acid from a heterologous signal peptide
  MOD_RES (22)..(22): Glu or any amino acid from a heterologous signal peptide
  MOD_RES (23)..(23): Ala or any amino acid from a heterologous signal peptide
XXXXXXXXXXXXXXXXXXXXXXXCTCSPSHPQDAFCNSDIVIRAKVVGKKLVKEGPFGTLVYTIKQMKMYRGFTKMPHVQYIHTEASESLCGLKLEVNKYQYLLTGRVYDGKMYTGLCNFVERWDQLTLSQRKGLNYRYHLGCNCKIKSCYYLPCFVTSKNECLWNDTLSNFGYPGYQSKHYACIRQKGGYCSWYRGWAPPDKSIINATDP

SEQ ID NO: 49 - protein, 211 aa, Artificial Sequence
  Description of Artificial Sequence: Synthetic polypeptide
  MOD_RES (1)..(1): Met or any amino acid from a heterologous signal peptide
  MOD_RES (2)..(2): Thr or any amino acid from a heterologous signal peptide
  MOD_RES (3)..(3): Pro or any amino acid from a heterologous signal peptide
  MOD_RES (4)..(4): Trp or any amino acid from a heterologous signal peptide
  MOD_RES (5)..(5): Leu or any amino acid from a heterologous signal peptide
  MOD_RES (6)..(6): Gly or any amino acid from a heterologous signal peptide
  MOD_RES (7)..(7): Leu or any amino acid from a heterologous signal peptide
  MOD_RES (8)..(8): Ile or any amino acid from a heterologous signal peptide
  MOD_RES (9)..(9): Val or any amino acid from a heterologous signal peptide
  MOD_RES (10)..(11): Leu or any amino acid from a heterologous signal peptide
  MOD_RES (12)..(12): Gly or any amino acid from a heterologous signal peptide
  MOD_RES (13)..(13): Ser or any amino acid from a heterologous signal peptide
  MOD_RES (14)..(14): Trp or any amino acid from a heterologous signal peptide
  MOD_RES (15)..(15): Ser or any amino acid from a heterologous signal peptide
  MOD_RES (16)..(16): Leu or any amino acid from a heterologous signal peptide
  MOD_RES (17)..(17): Gly or any amino acid from a heterologous signal peptide
  MOD_RES (18)..(18): Asp or any amino acid from a heterologous signal peptide
  MOD_RES (19)..(19): Trp or any amino acid from a heterologous signal peptide
  MOD_RES (20)..(20): Gly or any amino acid from a heterologous signal peptide
  MOD_RES (21)..(21): Ala or any amino acid from a heterologous signal peptide
  MOD_RES (22)..(22): Glu or any amino acid from a heterologous signal peptide
  MOD_RES (23)..(23): Ala or any amino acid from a heterologous signal peptide
XXXXXXXXXXXXXXXXXXXXXXXCTCSPSHPQDAFCNSDIVIRAKVVGKKLVKEGPFGTLVYTIKQMKMYRGFTKMPHVQYIHTEASESLCGLKLEVNKYQYLLTGRVYDGKMYTGLCNFVERWDQLTLSQRKGLNYRYHLGCNCKIKSCYYLPCFVTSKNECLWTDMLSNFTYPGYQSKHYACIRQKGGYCSWYRGWAPPDKSIINATDP

SEQ ID NO: 50 - protein, 211 aa, Artificial Sequence
  Description of Artificial Sequence: Synthetic polypeptide
  MOD_RES (1)..(1): Met or any amino acid from a heterologous signal peptide
  MOD_RES (2)..(2): Thr or any amino acid from a heterologous signal peptide
  MOD_RES (3)..(3): Pro or any amino acid from a heterologous signal peptide
  MOD_RES (4)..(4): Trp or any amino acid from a heterologous signal peptide
  MOD_RES (5)..(5): Leu or any amino acid from a heterologous signal peptide
  MOD_RES (6)..(6): Gly or any amino acid from a heterologous signal peptide
  MOD_RES (7)..(7): Leu or any amino acid from a heterologous signal peptide
  MOD_RES (8)..(8): Ile or any amino acid from a heterologous signal peptide
  MOD_RES (9)..(9): Val or any amino acid from a heterologous signal peptide
  MOD_RES (10)..(11): Leu or any amino acid from a heterologous signal peptide
  MOD_RES (12)..(12): Gly or any amino acid from a heterologous signal peptide
  MOD_RES (13)..(13): Ser or any amino acid from a heterologous signal peptide
  MOD_RES (14)..(14): Trp or any amino acid from a heterologous signal peptide
  MOD_RES (15)..(15): Ser or any amino acid from a heterologous signal peptide
  MOD_RES (16)..(16): Leu or any amino acid from a heterologous signal peptide
  MOD_RES (17)..(17): Gly or any amino acid from a heterologous signal peptide
  MOD_RES (18)..(18): Asp or any amino acid from a heterologous signal peptide
  MOD_RES (19)..(19): Trp or any amino acid from a heterologous signal peptide
  MOD_RES (20)..(20): Gly or any amino acid from a heterologous signal peptide
  MOD_RES (21)..(21): Ala or any amino acid from a heterologous signal peptide
  MOD_RES (22)..(22): Glu or any amino acid from a heterologous signal peptide
  MOD_RES (23)..(23): Ala or any amino acid from a heterologous signal peptide
XXXXXXXXXXXXXXXXXXXXXXXCTCSPSHPQDAFCNSDIVIRAKVVGKKLVKEGPFGTLVYTIKQMKMYRGFTKMPHVQYIHTEASESLCGLKLEVNKYQYLLTGRVYDGKMYTGLCNFVERWDQLTLSQRKGLNYRYHLGCNCKIKSCYYLPCFVTSKNECLWTDMLSNFGYPGYQSKNYTCIRQKGGYCSWYRGWAPPDKSIINATDP

SEQ ID NO: 51 - protein, 211 aa, Artificial Sequence
  Description of Artificial Sequence: Synthetic polypeptide
  MOD_RES (1)..(1): Met or any amino acid from a heterologous signal peptide
  MOD_RES (2)..(2): Thr or any amino acid from a heterologous signal peptide
  MOD_RES (3)..(3): Pro or any amino acid from a heterologous signal peptide
  MOD_RES (4)..(4): Trp or any amino acid from a heterologous signal peptide
  MOD_RES (5)..(5): Leu or any amino acid from a heterologous signal peptide
  MOD_RES (6)..(6): Gly or any amino acid from a heterologous signal peptide
  MOD_RES (7)..(7): Leu or any amino acid from a heterologous signal peptide
  MOD_RES (8)..(8): Ile or any amino acid from a heterologous signal peptide
  MOD_RES (9)..(9): Val or any amino acid from a heterologous signal peptide
  MOD_RES (10)..(11): Leu or any amino acid from a heterologous signal peptide
  MOD_RES (12)..(12): Gly or any amino acid from a heterologous signal peptide
  MOD_RES (13)..(13): Ser or any amino acid from a heterologous signal peptide
  MOD_RES (14)..(14): Trp or any amino acid from a heterologous signal peptide
  MOD_RES (15)..(15): Ser or any amino acid from a heterologous signal peptide
  MOD_RES (16)..(16): Leu or any amino acid from a heterologous signal peptide
  MOD_RES (17)..(17): Gly or any amino acid from a heterologous signal peptide
  MOD_RES (18)..(18): Asp or any amino acid from a heterologous signal peptide
  MOD_RES (19)..(19): Trp or any amino acid from a heterologous signal peptide
  MOD_RES (20)..(20): Gly or any amino acid from a heterologous signal peptide
  MOD_RES (21)..(21): Ala or any amino acid from a heterologous signal peptide
  MOD_RES (22)..(22): Glu or any amino acid from a heterologous signal peptide
  MOD_RES (23)..(23): Ala or any amino acid from a heterologous signal peptide
XXXXXXXXXXXXXXXXXXXXXXXCTCSPSHPQDAFCNSDIVIRAKVVGKKLVKEGPFGTLVYTIKQMKMYRGFTKMPHVQYIHTEASESLCGLKLEVNKYQYLLTGRVYDGKMYTGLCNFVERWDQLTLSQRKGLNYRYHLGCNCKIKSCYYLPCFVTSKNECLWTDMLSNFGYPGYQSKHYACINQTGGYCSWYRGWAPPDKSIINATDP

SEQ ID NO: 52 - protein, 211 aa, Artificial Sequence
  Description of Artificial Sequence: Synthetic polypeptide
  MOD_RES (1)..(1): Met or any amino acid from a heterologous signal peptide
  MOD_RES (2)..(2): Thr or any amino acid from a heterologous signal peptide
  MOD_RES (3)..(3): Pro or any amino acid from a heterologous signal peptide
  MOD_RES (4)..(4): Trp or any amino acid from a heterologous signal peptide
  MOD_RES (5)..(5): Leu or any amino acid from a heterologous signal peptide
  MOD_RES (6)..(6): Gly or any amino acid from a heterologous signal peptide
  MOD_RES (7)..(7): Leu or any amino acid from a heterologous signal peptide
  MOD_RES (8)..(8): Ile or any amino acid from a heterologous signal peptide
  MOD_RES (9)..(9): Val or any amino acid from a heterologous signal peptide
  MOD_RES (10)..(11): Leu or any amino acid from a heterologous signal peptide
  MOD_RES (12)..(12): Gly or any amino acid from a heterologous signal peptide
  MOD_RES (13)..(13): Ser or any amino acid from a heterologous signal peptide
  MOD_RES (14)..(14): Trp or any amino acid from a heterologous signal peptide
  MOD_RES (15)..(15): Ser or any amino acid from a heterologous signal peptide
  MOD_RES (16)..(16): Leu or any amino acid from a heterologous signal peptide
  MOD_RES (17)..(17): Gly or any amino acid from a heterologous signal peptide
  MOD_RES (18)..(18): Asp or any amino acid from a heterologous signal peptide
  MOD_RES (19)..(19): Trp or any amino acid from a heterologous signal peptide
  MOD_RES (20)..(20): Gly or any amino acid from a heterologous signal peptide
  MOD_RES (21)..(21): Ala or any amino acid from a heterologous signal peptide
  MOD_RES (22)..(22): Glu or any amino acid from a heterologous signal peptide
  MOD_RES (23)..(23): Ala or any amino acid from a heterologous signal peptide
XXXXXXXXXXXXXXXXXXXXXXXCTCSPSHPQDAFCNSDIVIRAKVVGKKLVKEGPFGTLVYTIKQMKMYRGFTKMPHVQYIHTEASESLCGLKLEVNKYQYLLTGRVYDGKMYTGLCNFVERWDQLTLSQRKGLNYRYHLGCNCKIKSCYYLPCFVTSKNECLWTDMLSNFGYPGYQSKHYACIRQKGGYCSWYRGWAPNDTSIINATDP

SEQ ID NO: 53 - protein, 211 aa, Artificial Sequence; identical to SEQ ID NO: 15
  Description of Artificial Sequence: Synthetic polypeptide
  MOD_RES (1)..(1): Met or any amino acid from a heterologous signal peptide
  MOD_RES (2)..(2): Thr or any amino acid from a heterologous signal peptide
  MOD_RES (3)..(3): Pro or any amino acid from a heterologous signal peptide
  MOD_RES (4)..(4): Trp or any amino acid from a heterologous signal peptide
  MOD_RES (5)..(5): Leu or any amino acid from a heterologous signal peptide
  MOD_RES (6)..(6): Gly or any amino acid from a heterologous signal peptide
  MOD_RES (7)..(7): Leu or any amino acid from a heterologous signal peptide
  MOD_RES (8)..(8): Ile or any amino acid from a heterologous signal peptide
  MOD_RES (9)..(9): Val or any amino acid from a heterologous signal peptide
  MOD_RES (10)..(11): Leu or any amino acid from a heterologous signal peptide
  MOD_RES (12)..(12): Gly or any amino acid from a heterologous signal peptide
  MOD_RES (13)..(13): Ser or any amino acid from a heterologous signal peptide
  MOD_RES (14)..(14): Trp or any amino acid from a heterologous signal peptide
  MOD_RES (15)..(15): Ser or any amino acid from a heterologous signal peptide
  MOD_RES (16)..(16): Leu or any amino acid from a heterologous signal peptide
  MOD_RES (17)..(17): Gly or any amino acid from a heterologous signal peptide
  MOD_RES (18)..(18): Asp or any amino acid from a heterologous signal peptide
  MOD_RES (19)..(19): Trp or any amino acid from a heterologous signal peptide
  MOD_RES (20)..(20): Gly or any amino acid from a heterologous signal peptide
  MOD_RES (21)..(21): Ala or any amino acid from a heterologous signal peptide
  MOD_RES (22)..(22): Glu or any amino acid from a heterologous signal peptide
  MOD_RES (23)..(23): Ala or any amino acid from a heterologous signal peptide

SEQ ID NO: 54 - protein, 211 aa, Artificial Sequence
  Description of Artificial Sequence: Synthetic polypeptide
  MOD_RES (1)..(1): Met or any amino acid from a heterologous signal peptide
  MOD_RES (2)..(2): Thr or any amino acid from a heterologous signal peptide
  MOD_RES (3)..(3): Pro or any amino acid from a heterologous signal peptide
  MOD_RES (4)..(4): Trp or any amino acid from a heterologous signal peptide
  MOD_RES (5)..(5): Leu or any amino acid from a heterologous signal peptide
  MOD_RES (6)..(6): Gly or any amino acid from a heterologous signal peptide
  MOD_RES (7)..(7): Leu or any amino acid from a heterologous signal peptide
  MOD_RES (8)..(8): Ile or any amino acid from a heterologous signal peptide
  MOD_RES (9)..(9): Val or any amino acid from a heterologous signal peptide
  MOD_RES (10)..(11): Leu or any amino acid from a heterologous signal peptide
  MOD_RES (12)..(12): Gly or any amino acid from a heterologous signal peptide
  MOD_RES (13)..(13): Ser or any amino acid from a heterologous signal peptide
  MOD_RES (14)..(14): Trp or any amino acid from a heterologous signal peptide
  MOD_RES (15)..(15): Ser or any amino acid from a heterologous signal peptide
  MOD_RES (16)..(16): Leu or any amino acid from a heterologous signal peptide
  MOD_RES (17)..(17): Gly or any amino acid from a heterologous signal peptide
  MOD_RES (18)..(18): Asp or any amino acid from a heterologous signal peptide
  MOD_RES (19)..(19): Trp or any amino acid from a heterologous signal peptide
  MOD_RES (20)..(20): Gly or any amino acid from a heterologous signal peptide
  MOD_RES (21)..(21): Ala or any amino acid from a heterologous signal peptide
  MOD_RES (22)..(22): Glu or any amino acid from a heterologous signal peptide
  MOD_RES (23)..(23): Ala or any amino acid from a heterologous signal peptide
XXXXXXXXXXXXXXXXXXXXXXXCTCSPSHPQDAFCNSDIVIRAKVVGKKNVTEGPFGTLVYTIKQMKMYRGFTKMPHVQYIHTEASESLCGLKLEVNKYQYLLTGRVYDGKMYTGLCNFVERWDQLTLSQRKGLNYRYHLGCNCKIKSCYYLPCFVTSKNECLWTDMLSNFGYPGYQSKHYACIRQKGGYCSWYRGWAPPDKSIINATDP

SEQ ID NO: 55 - protein, 211 aa, Artificial Sequence
  Description of Artificial Sequence: Synthetic polypeptide
  MOD_RES (1)..(1): Met or any amino acid from a heterologous signal peptide
  MOD_RES (2)..(2): Thr or any amino acid from a heterologous signal peptide
  MOD_RES (3)..(3): Pro or any amino acid from a heterologous signal peptide
  MOD_RES (4)..(4): Trp or any amino acid from a heterologous signal peptide
  MOD_RES (5)..(5): Leu or any amino acid from a heterologous signal peptide
  MOD_RES (6)..(6): Gly or any amino acid from a heterologous signal peptide
  MOD_RES (7)..(7): Leu or any amino acid from a heterologous signal peptide
  MOD_RES (8)..(8): Ile or any amino acid from a heterologous signal peptide
  MOD_RES (9)..(9): Val or any amino acid from a heterologous signal peptide
  MOD_RES (10)..(11): Leu or any amino acid from a heterologous signal peptide
  MOD_RES (12)..(12): Gly or any amino acid from a heterologous signal peptide
  MOD_RES (13)..(13): Ser or any amino acid from a heterologous signal peptide
  MOD_RES (14)..(14): Trp or any amino acid from a heterologous signal peptide
  MOD_RES (15)..(15): Ser or any amino acid from a heterologous signal peptide
  MOD_RES (16)..(16): Leu or any amino acid from a heterologous signal peptide
  MOD_RES (17)..(17): Gly or any amino acid from a heterologous signal peptide
  MOD_RES (18)..(18): Asp or any amino acid from a heterologous signal peptide
  MOD_RES (19)..(19): Trp or any amino acid from a heterologous signal peptide
  MOD_RES (20)..(20): Gly or any amino acid from a heterologous signal peptide
  MOD_RES (21)..(21): Ala or any amino acid from a heterologous signal peptide
  MOD_RES (22)..(22): Glu or any amino acid from a heterologous signal peptide
  MOD_RES (23)..(23): Ala or any amino acid from a heterologous signal peptide
XXXXXXXXXXXXXXXXXXXXXXXCTCSPSHPQDAFCNSDIVIRAKVVGKKLVKEGPFGTLVYTIKQMKMYRGFTKMPHVQYIHTEASESLCGLKLEVNKYQYLLTGRVYDGKMYTGLCNFVERWDQLTLSQRKGLNYRYHLGCNCKIKSCYYLPCFVTSKNECLWTDMLSNFGYPGYQSKHYACIRQKGGYCSWYRGWAPPDKSIINYTDP

SEQ ID NO: 56 - protein, 211 aa, Artificial Sequence
  Description of Artificial Sequence: Synthetic polypeptide
  MOD_RES (1)..(1): Met or any amino acid from a heterologous signal peptide
  MOD_RES (2)..(2): Thr or any amino acid from a heterologous signal peptide
  MOD_RES (3)..(3): Pro or any amino acid from a heterologous signal peptide
  MOD_RES (4)..(4): Trp or any amino acid from a heterologous signal peptide
  MOD_RES (5)..(5): Leu or any amino acid from a heterologous signal peptide
  MOD_RES (6)..(6): Gly or any amino acid from a heterologous signal peptide
  MOD_RES (7)..(7): Leu or any amino acid from a heterologous signal peptide
  MOD_RES (8)..(8): Ile or any amino acid from a heterologous signal peptide
  MOD_RES (9)..(9): Val or any amino acid from a heterologous signal peptide
  MOD_RES (10)..(11): Leu or any amino acid from a heterologous signal peptide
  MOD_RES (12)..(12): Gly or any amino acid from a heterologous signal peptide
  MOD_RES (13)..(13): Ser or any amino acid from a heterologous signal peptide
  MOD_RES (14)..(14): Trp or any amino acid from a heterologous signal peptide
  MOD_RES (15)..(15): Ser or any amino acid from a heterologous signal peptide
  MOD_RES (16)..(16): Leu or any amino acid from a heterologous signal peptide
  MOD_RES (17)..(17): Gly or any amino acid from a heterologous signal peptide
  MOD_RES (18)..(18): Asp or any amino acid from a heterologous signal peptide
  MOD_RES (19)..(19): Trp or any amino acid from a heterologous signal peptide
  MOD_RES (20)..(20): Gly or any amino acid from a heterologous signal peptide
  MOD_RES (21)..(21): Ala or any amino acid from a heterologous signal peptide
  MOD_RES (22)..(22): Glu or any amino acid from a heterologous signal peptide
  MOD_RES (23)..(23): Ala or any amino acid from a heterologous signal peptide
XXXXXXXXXXXXXXXXXXXXXXXCTCSPSHPQDAFCNSDIVIRAKVVGKKLVKEGPFGTLVYTIKQMKMYRGFTKMPHVQYIHTEASESLCGLKLEVNKYQYLLTGRVYDGKMYTGLCNFVERWDQLTLSQRKGLNYRYHLGCNCKIKSCYYLPCFVTSKNECLWTDMLSNFGYPGYQSKHYACIRQKGGYCSWYRGWAPPDKSIINVTDP

SEQ ID NO: 57 - protein, 188 aa, Homo sapiens
  huTIMP3(K45S, F57N, I205F, A208G)
CTCSPSHPQDAFCNSDIVIRASVVGKKLVKEGPNGTLVYTIKQMKMYRGFTKMPHVQYIHTEASESLCGLKLEVNKYQYLLTGRVYDGKMYTGLCNFVERWDQLTLSQRKGLNYRYHLGCNCKIKSCYYLPCFVTSKNECLWTDMLSNFGYPGYQSKHYACIRQKGGYCSWYRGWAPPDKSFINGTDP

SEQ ID NO: 58 - protein, 188 aa, Homo sapiens
  huTIMP3(K45S, F57N, A208G)
CTCSPSHPQDAFCNSDIVIRASVVGKKLVKEGPNGTLVYTIKQMKMYRGFTKMPHVQYIHTEASESLCGLKLEVNKYQYLLTGRVYDGKMYTGLCNFVERWDQLTLSQRKGLNYRYHLGCNCKIKSCYYLPCFVTSKNECLWTDMLSNFGYPGYQSKHYACIRQKGGYCSWYRGWAPPDKSIINGTDP

SEQ ID NO: 59 - protein, 188 aa, Homo sapiens
  huTIMP3(K45S, F57N, I205Y)
CTCSPSHPQDAFCNSDIVIRASVVGKKLVKEGPNGTLVYTIKQMKMYRGFTKMPHVQYIHTEASESLCGLKLEVNKYQYLLTGRVYDGKMYTGLCNFVERWDQLTLSQRKGLNYRYHLGCNCKIKSCYYLPCFVTSKNECLWTDMLSNFGYPGYQSKHYACIRQKGGYCSWYRGWAPPDKSYINATDP

SEQ ID NO: 60 - protein, 188 aa, Homo sapiens
  huTIMP3(K45S, F57N, I205Y, A208G)
CTCSPSHPQDAFCNSDIVIRASVVGKKLVKEGPNGTLVYTIKQMKMYRGFTKMPHVQYIHTEASESLCGLKLEVNKYQYLLTGRVYDGKMYTGLCNFVERWDQLTLSQRKGLNYRYHLGCNCKIKSCYYLPCFVTSKNECLWTDMLSNFGYPGYQSKHYACIRQKGGYCSWYRGWAPPDKSYINGTDP

SEQ ID NO: 61 - protein, 188 aa, Homo sapiens
  huTIMP3(K45N,V47T,F57N,K75N,P77T,K94N,E96T,R138T,G173T)
CTCSPSHPQDAFCNSDIVIRANVTGKKLVKEGPNGTLVYTIKQMKMYRGFTNMTHVQYIHTEASESLCGLNLTVNKYQYLLTGRVYDGKMYTGLCNFVERWDQLTLSQRKGLNYTYHLGCNCKIKSCYYLPCFVTSKNECLWTDMLSNFTYPGYQSKHYACIRQKGGYCSWYRGWAPPDKSIINATDP

SEQ ID NO: 62 - protein, 188 aa, Homo sapiens
  huTIMP3(K45N,V47T,F57N,K94N,E96T,R138T,G173T)
CTCSPSHPQDAFCNSDIVIRANVTGKKLVKEGPNGTLVYTIKQMKMYRGFTKMPHVQYIHTEASESLCGLNLTVNKYQYLLTGRVYDGKMYTGLCNFVERWDQLTLSQRKGLNYTYHLGCNCKIKSCYYLPCFVTSKNECLWTDMLSNFTYPGYQSKHYACIRQKGGYCSWYRGWAPPDKSIINATDP

SEQ ID NO: 63 - protein, 188 aa, Homo sapiens
  huTIMP3(K45N,V47T,K50N,V52T,F57N,V97N,K99T)
CTCSPSHPQDAFCNSDIVIRANVTGKNLTKEGPNGTLVYTIKQMKMYRGFTKMPHVQYIHTEASESLCGLKLENNTYQYLLTGRVYDGKMYTGLCNFVERWDQLTLSQRKGLNYRYHLGCNCKIKSCYYLPCFVTSKNECLWTDMLSNFGYPGYQSKHYACIRQKGGYCSWYRGWAPPDKSIINATDP

SEQ ID NO: 64 - protein, 188 aa, Homo sapiens
  huTIMP3(K45S,K50N,V52T,F57N,V97N,K99T,R186N,K188T)
CTCSPSHPQDAFCNSDIVIRASVVGKNLTKEGPNGTLVYTIKQMKMYRGFTKMPHVQYIHTEASESLCGLKLENNTYQYLLTGRVYDGKMYTGLCNFVERWDQLTLSQRKGLNYRYHLGCNCKIKSCYYLPCFVTSKNECLWTDMLSNFGYPGYQSKHYACINQTGGYCSWYRGWAPPDKSIINATDP

SEQ ID NO: 65 - protein, 188 aa, Homo sapiens
  huTIMP3(K45S,F57N,K94N,E96T,D110N,K112T,R138T,G173T)
CTCSPSHPQDAFCNSDIVIRASVVGKKLVKEGPNGTLVYTIKQMKMYRGFTKMPHVQYIHTEASESLCGLNLTVNKYQYLLTGRVYNGTMYTGLCNFVERWDQLTLSQRKGLNYTYHLGCNCKIKSCYYLPCFVTSKNECLWTDMLSNFTYPGYQSKHYACIRQKGGYCSWYRGWAPPDKSIINATDP

SEQ ID NO: 66 - protein, 188 aa, Homo sapiens
  huTIMP3(K45S,F57N,T63N,K65T,K94N,E96T,G173T)
CTCSPSHPQDAFCNSDIVIRASVVGKKLVKEGPNGTLVYNITQMKMYRGFTKMPHVQYIHTEASESLCGLNLTVNKYQYLLTGRVYDGKMYTGLCNFVERWDQLTLSQRKGLNYRYHLGCNCKIKSCYYLPCFVTSKNECLWTDMLSNFTYPGYQSKHYACIRQKGGYCSWYRGWAPPDKSIINATDP

SEQ ID NO: 67 - protein, 188 aa, Homo sapiens
  huTIMP3(K45N,V47T,K50N,V52T,F57N,V97N,K99T,R138T,R186N,K188T)
CTCSPSHPQDAFCNSDIVIRANVTGKNLTKEGPNGTLVYTIKQMKMYRGFTKMPHVQYIHTEASESLCGLKLENNTYQYLLTGRVYDGKMYTGLCNFVERWDQLTLSQRKGLNYTYHLGCNCKIKSCYYLPCFVTSKNECLWTDMLSNFGYPGYQSKHYACINQTGGYCSWYRGWAPPDKSIINATDP

SEQ ID NO: 68 - protein, 188 aa, Homo sapiens
  huTIMP3(K45S,F57N,T63N,K65T,K94N,E96T,Q126N,R138T)
CTCSPSHPQDAFCNSDIVIRASVVGKKLVKEGPNGTLVYNITQMKMYRGFTKMPHVQYIHTEASESLCGLNLTVNKYQYLLTGRVYDGKMYTGLCNFVERWDNLTLSQRKGLNYTYHLGCNCKIKSCYYLPCFVTSKNECLWTDMLSNFGYPGYQSKHYACIRQKGGYCSWYRGWAPPDKSIINATDP

SEQ ID NO: 69 - protein, 188 aa, Homo sapiens
  huTIMP3(K45N,V47T,K50N,V52T,F57N,V97N,K99T,R186N,K188T)
CTCSPSHPQDAFCNSDIVIRANVTGKNLTKEGPNGTLVYTIKQMKMYRGFTKMPHVQYIHTEASESLCGLKLENNTYQYLLTGRVYDGKMYTGLCNFVERWDQLTLSQRKGLNYRYHLGCNCKIKSCYYLPCFVTSKNECLWTDMLSNFGYPGYQSKHYACINQTGGYCSWYRGWAPPDKSIINATDP

SEQ ID NO: 70 - protein, 188 aa, Homo sapiens
  huTIMP3(K45N,V47T,K50N,V52T,V97N,K99T,R138T,R186N,K188T)
CTCSPSHPQDAFCNSDIVIRANVTGKNLTKEGPFGTLVYTIKQMKMYRGFTKMPHVQYIHTEASESLCGLKLENNTYQYLLTGRVYDGKMYTGLCNFVERWDQLTLSQRKGLNYTYHLGCNCKIKSCYYLPCFVTSKNECLWTDMLSNFGYPGYQSKHYACINQTGGYCSWYRGWAPPDKSIINATDP

SEQ ID NO: 71 - protein, 188 aa, Homo sapiens
  huTIMP3(K45S,F57N,H78N,Q80T,K94N,E96T,R138T,G173T)
CTCSPSHPQDAFCNSDIVIRASVVGKKLVKEGPNGTLVYTIKQMKMYRGFTKMPNVTYIHTEASESLCGLNLTVNKYQYLLTGRVYDGKMYTGLCNFVERWDQLTLSQRKGLNYTYHLGCNCKIKSCYYLPCFVTSKNECLWTDMLSNFTYPGYQSKHYACIRQKGGYCSWYRGWAPPDKSIINATDP

SEQ ID NO: 72 - protein, 188 aa, Homo sapiens
  huTIMP3(K45S,F57N,K75N,P77T,K94N,E96T,R138T,G173T)
CTCSPSHPQDAFCNSDIVIRASVVGKKLVKEGPNGTLVYTIKQMKMYRGFTNMTHVQYIHTEASESLCGLNLTVNKYQYLLTGRVYDGKMYTGLCNFVERWDQLTLSQRKGLNYTYHLGCNCKIKSCYYLPCFVTSKNECLWTDMLSNFTYPGYQSKHYACIRQKGGYCSWYRGWAPPDKSIINATDP

SEQ ID NO: 73 - protein, 188 aa, Homo sapiens
  huTIMP3(K45N,V47T,K50N,V52T,V97N,K99T,G173T,R186N,K188T)
CTCSPSHPQDAFCNSDIVIRANVTGKNLTKEGPFGTLVYTIKQMKMYRGFTKMPHVQYIHTEASESLCGLKLENNTYQYLLTGRVYDGKMYTGLCNFVERWDQLTLSQRKGLNYRYHLGCNCKIKSCYYLPCFVTSKNECLWTDMLSNFTYPGYQSKHYACINQTGGYCSWYRGWAPPDKSIINATDP

SEQ ID NO: 74 - protein, 188 aa, Homo sapiens
  huTIMP3(K45E,F57N,Q126N,R138T,G173T)
CTCSPSHPQDAFCNSDIVIRAEVVGKKLVKEGPNGTLVYTIKQMKMYRGFTKMPHVQYIHTEASESLCGLKLEVNKYQYLLTGRVYDGKMYTGLCNFVERWDNLTLSQRKGLNYTYHLGCNCKIKSCYYLPCFVTSKNECLWTDMLSNFTYPGYQSKHYACIRQKGGYCSWYRGWAPPDKSIINATDP

SEQ ID NO: 75 - protein, 188 aa, Homo sapiens
  huTIMP3(K45S,F57N,T63N,K65T,K94N,E96T,R138T,G173T)
CTCSPSHPQDAFCNSDIVIRASVVGKKLVKEGPNGTLVYNITQMKMYRGFTKMPHVQYIHTEASESLCGLNLTVNKYQYLLTGRVYDGKMYTGLCNFVERWDQLTLSQRKGLNYTYHLGCNCKIKSCYYLPCFVTSKNECLWTDMLSNFTYPGYQSKHYACIRQKGGYCSWYRGWAPPDKSIINATDP

SEQ ID NO: 76 - protein, 188 aa, Homo sapiens
  huTIMP3(K45S,K50N,V52T,F57N,V97N,K99T,R138T,R186N,K188T)
CTCSPSHPQDAFCNSDIVIRASVVGKNLTKEGPNGTLVYTIKQMKMYRGFTKMPHVQYIHTEASESLCGLKLENNTYQYLLTGRVYDGKMYTGLCNFVERWDQLTLSQRKGLNYTYHLGCNCKIKSCYYLPCFVTSKNECLWTDMLSNFGYPGYQSKHYACINQTGGYCSWYRGWAPPDKSIINATDP

SEQ ID NO: 77 - protein, 188 aa, Homo sapiens
  huTIMP3(K45S.K50N,V52T,F57N,V97N,K99T,G173T,R186N,K188T)
CTCSPSHPQDAFCNSDIVIRASVVGKNLTKEGPNGTLVYTIKQMKMYRGFTKMPHVQYIHTEASESLCGLKLENNTYQYLLTGRVYDGKMYTGLCNFVERWDQLTLSQRKGLNYRYHLGCNCKIKSCYYLPCFVTSKNECLWTDMLSNFTYPGYQSKHYACINQTGGYCSWYRGWAPPDKSIINATDP

SEQ ID NO: 78 - protein, 188 aa, Homo sapiens
  huTIMP3(K45N,V47T, F57N, K94N,E96T, G173T, R186N,K188T)
CTCSPSHPQDAFCNSDIVIRANVTGKKLVKEGPNGTLVYTIKQMKMYRGFTKMPHVQYIHTEASESLCGLNLTVNKYQYLLTGRVYDGKMYTGLCNFVERWDQLTLSQRKGLNYRYHLGCNCKIKSCYYLPCFVTSKNECLWTDMLSNFTYPGYQSKHYACINQTGGYCSWYRGWAPPDKSIINATDP

SEQ ID NO: 79 - protein, 188 aa, Homo sapiens
  huTIMP3(K45N,V47T, F57N, K94N,E96T, D110N,K112T, R186N,K188T)
CTCSPSHPQDAFCNSDIVIRANVTGKKLVKEGPNGTLVYTIKQMKMYRGFTKMPHVQYIHTEASESLCGLNLTVNKYQYLLTGRVYNGTMYTGLCNFVERWDQLTLSQRKGLNYRYHLGCNCKIKSCYYLPCFVTSKNECLWTDMLSNFGYPGYQSKHYACINQTGGYCSWYRGWAPPDKSIINATDP

SEQ ID NO: 80 - protein, 188 aa, Homo sapiens
  huTIMP3(K45N,V47T, F57N, V97N,K99T, R138T, G173T)
CTCSPSHPQDAFCNSDIVIRANVTGKKLVKEGPNGTLVYTIKQMKMYRGFTKMPHVQYIHTEASESLCGLKLENNTYQYLLTGRVYDGKMYTGLCNFVERWDQLTLSQRKGLNYTYHLGCNCKIKSCYYLPCFVTSKNECLWTDMLSNFTYPGYQSKHYACIRQKGGYCSWYRGWAPPDKSIINATDP

SEQ ID NO: 81 - protein, 188 aa, Homo sapiens
  huTIMP3(K45N,V47T, F57N, K99E G173T, R186N,K188T)
CTCSPSHPQDAFCNSDIVIRANVTGKKLVKEGPNGTLVYTIKQMKMYRGFTKMPHVQYIHTEASESLCGLKLEVNEYQYLLTGRVYDGKMYTGLCNFVERWDQLTLSQRKGLNYRYHLGCNCKIKSCYYLPCFVTSKNECLWTDMLSNFTYPGYQSKHYACINQTGGYCSWYRGWAPPDKSIINATDP

SEQ ID NO: 82 - protein, 188 aa, Homo sapiens
  huTIMP3(K45E, K49E, F57N, K94N,E96T, D110N,K112T, G173T, R186N,K188T)
CTCSPSHPQDAFCNSDIVIRAEVVGEKLVKEGPNGTLVYTIKQMKMYRGFTKMPHVQYIHTEASESLCGLNLTVNKYQYLLTGRVYNGTMYTGLCNFVERWDQLTLSQRKGLNYRYHLGCNCKIKSCYYLPCFVTSKNECLWTDMLSNFTYPGYQSKHYACINQTGGYCSWYRGWAPPDKSIINATDP

SEQ ID NO: 83 - protein, 188 aa, Homo sapiens
  huTIMP3(K50N,V52T, K94N,E96T, R138T, G173T)
CTCSPSHPQDAFCNSDIVIRAKVVGKNLTKEGPFGTLVYTIKQMKMYRGFTKMPHVQYIHTEASESLCGLNLTVNKYQYLLTGRVYDGKMYTGLCNFVERWDQLTLSQRKGLNYTYHLGCNCKIKSCYYLPCFVTSKNECLWTDMLSNFTYPGYQSKHYACIRQKGGYCSWYRGWAPPDKSIINATDP

SEQ ID NO: 84 - protein, 188 aa, Homo sapiens
  huTIMP3(K45E, K50N,V52T, K94N,E96T, D110N,K112T, R138T, G173T)
CTCSPSHPQDAFCNSDIVIRAEVVGKNLTKEGPFGTLVYTIKQMKMYRGFTKMPHVQYIHTEASESLCGLNLTVNKYQYLLTGRVYNGTMYTGLCNFVERWDQLTLSQRKGLNYTYHLGCNCKIKSCYYLPCFVTSKNECLWTDMLSNFTYPGYQSKHYACIRQKGGYCSWYRGWAPPDKSIINATDP

SEQ ID NO: 85 - protein, 188 aa, Homo sapiens
  huTIMP3(K50N,V52T, K94N,E96T, R138T, G173T, R186N,K188T)
CTCSPSHPQDAFCNSDIVIRAKVVGKNLTKEGPFGTLVYTIKQMKMYRGFTKMPHVQYIHTEASESLCGLNLTVNKYQYLLTGRVYDGKMYTGLCNFVERWDQLTLSQRKGLNYTYHLGCNCKIKSCYYLPCFVTSKNECLWTDMLSNFTYPGYQSKHYACINQTGGYCSWYRGWAPPDKSIINATDP

SEQ ID NO: 86 - protein, 188 aa, Homo sapiens
  huTIMP3(K45E, F57N ,T63N,K65T, K94N,E96T ,G173T, R186N,K188T)
CTCSPSHPQDAFCNSDIVIRAEVVGKKLVKEGPNGTLVYNITQMKMYRGFTKMPHVQYIHTEASESLCGLNLTVNKYQYLLTGRVYDGKMYTGLCNFVERWDQLTLSQRKGLNYRYHLGCNCKIKSCYYLPCFVTSKNECLWTDMLSNFTYPGYQSKHYACINQTGGYCSWYRGWAPPDKSIINATDP

SEQ ID NO: 87 - protein, 188 aa, Homo sapiens
  huTIMP3(K45N,V47T, F57N, K94N,E96T, D110N,K112T, G173T, R186Q,K188Q)
CTCSPSHPQDAFCNSDIVIRANVTGKKLVKEGPNGTLVYTIKQMKMYRGFTKMPHVQYIHTEASESLCGLNLTVNKYQYLLTGRVYNGTMYTGLCNFVERWDQLTLSQRKGLNYRYHLGCNCKIKSCYYLPCFVTSKNECLWTDMLSNFTYPGYQSKHYACIQQQGGYCSWYRGWAPPDKSIINATDP

SEQ ID NO: 88 - protein, 188 aa, Homo sapiens
  HuTIMP3(K45S, F57N, K94N, E96T, R138T, G173T)
CTCSPSHPQDAFCNSDIVIRASVVGKKLVKEGPNGTLVYTIKQMKMYRGFTKMPHVQYIHTEASESLCGLNLTVNKYQYLLTGRVYDGKMYTGLCNFVERWDQLTLSQRKGLNYTYHLGCNCKIKSCYYLPCFVTSKNECLWTDMLSNFTYPGYQSKHYACIRQKGGYCSWYRGWAPPDKSIINATDP

SEQ ID NO: 89 - protein, 188 aa, Homo sapiens
  HuTIMP3(K45E, F57N, K94N, E96T, R138T, G173T)
CTCSPSHPQDAFCNSDIVIRAEVVGKKLVKEGPNGTLVYTIKQMKMYRGFTKMPHVQYIHTEASESLCGLNLTVNKYQYLLTGRVYDGKMYTGLCNFVERWDQLTLSQRKGLNYTYHLGCNCKIKSCYYLPCFVTSKNECLWTDMLSNFTYPGYQSKHYACIRQKGGYCSWYRGWAPPDKSIINATDP

SEQ ID NO: 90 - protein, 188 aa, Homo sapiens
  HuTIMP3(K45E, F57N, K94N, E96T, D110N, K112T, R138T, G173T)
CTCSPSHPQDAFCNSDIVIRAEVVGKKLVKEGPNGTLVYTIKQMKMYRGFTKMPHVQYIHTEASESLCGLNLTVNKYQYLLTGRVYNGTMYTGLCNFVERWDQLTLSQRKGLNYTYHLGCNCKIKSCYYLPCFVTSKNECLWTDMLSNFTYPGYQSKHYACIRQKGGYCSWYRGWAPPDKSIINATDP

SEQ ID NO: 91 - protein, 188 aa, Homo sapiens
  HuTIMP3(K45E, F57N, K94N, E96T, R138T, G173T, R186Q, K188Q)
CTCSPSHPQDAFCNSDIVIRAEVVGKKLVKEGPNGTLVYTIKQMKMYRGFTKMPHVQYIHTEASESLCGLNLTVNKYQYLLTGRVYDGKMYTGLCNFVERWDQLTLSQRKGLNYTYHLGCNCKIKSCYYLPCFVTSKNECLWTDMLSNFTYPGYQSKHYACIQQQGGYCSWYRGWAPPDKSIINATDP

SEQ ID NO: 92 - protein, 188 aa, Homo sapiens
  HuTIMP3(K45E, F57N, K94N, E96T, R138T, G173T, R186E)
CTCSPSHPQDAFCNSDIVIRAEVVGKKLVKEGPNGTLVYTIKQMKMYRGFTKMPHVQYIHTEASESLCGLNLTVNKYQYLLTGRVYDGKMYTGLCNFVERWDQLTLSQRKGLNYTYHLGCNCKIKSCYYLPCFVTSKNECLWTDMLSNFTYPGYQSKHYACIEQKGGYCSWYRGWAPPDKSIINATDP

SEQ ID NO: 93 - protein, 188 aa, Homo sapiens
  HuTIMP3(K45E, F57N, K94N, E96T, R138T, G173T, K188E)
CTCSPSHPQDAFCNSDIVIRAEVVGKKLVKEGPNGTLVYTIKQMKMYRGFTKMPHVQYIHTEASESLCGLNLTVNKYQYLLTGRVYDGKMYTGLCNFVERWDQLTLSQRKGLNYTYHLGCNCKIKSCYYLPCFVTSKNECLWTDMLSNFTYPGYQSKHYACIRQEGGYCSWYRGWAPPDKSIINATDP

SEQ ID NO: 94 - protein, 188 aa, Homo sapiens
  HuTIMP3(K45E, F57N, K94N, E96T, R138T, G173T, R186N, K188T)
CTCSPSHPQDAFCNSDIVIRAEVVGKKLVKEGPNGTLVYTIKQMKMYRGFTKMPHVQYIHTEASESLCGLNLTVNKYQYLLTGRVYDGKMYTGLCNFVERWDQLTLSQRKGLNYTYHLGCNCKIKSCYYLPCFVTSKNECLWTDMLSNFTYPGYQSKHYACINQTGGYCSWYRGWAPPDKSIINATDP

SEQ ID NO: 95 - protein, 188 aa, Homo sapiens; identical to SEQ ID NO: 84
  HuTIMP3(K45E, K50N, V52T, K94N, E96T, D110N, K112T, R138T, G173T)

SEQ ID NO: 96 - protein, 188 aa, Homo sapiens
  HuTIMP3(K45E, K50N, V52T, K94N, E96T, R138T, G173T, K188E)
CTCSPSHPQDAFCNSDIVIRAEVVGKNLTKEGPFGTLVYTIKQMKMYRGFTKMPHVQYIHTEASESLCGLNLTVNKYQYLLTGRVYDGKMYTGLCNFVERWDQLTLSQRKGLNYTYHLGCNCKIKSCYYLPCFVTSKNECLWTDMLSNFTYPGYQSKHYACIRQEGGYCSWYRGWAPPDKSIINATDP

SEQ ID NO: 97 - protein, 188 aa, Homo sapiens
  HuTIMP3(K50N, V52T, F57N, K94N, E96T, R138T, G173T)
CTCSPSHPQDAFCNSDIVIRAKVVGKNLTKEGPNGTLVYTIKQMKMYRGFTKMPHVQYIHTEASESLCGLNLTVNKYQYLLTGRVYDGKMYTGLCNFVERWDQLTLSQRKGLNYTYHLGCNCKIKSCYYLPCFVTSKNECLWTDMLSNFTYPGYQSKHYACIRQKGGYCSWYRGWAPPDKSIINATDP

SEQ ID NO: 98 - protein, 188 aa, Homo sapiens
  HuTIMP3(K50N, V52T, F57N, K94N, E96T, D110N, K112T, R138T)
CTCSPSHPQDAFCNSDIVIRAKVVGKNLTKEGPNGTLVYTIKQMKMYRGFTKMPHVQYIHTEASESLCGLNLTVNKYQYLLTGRVYNGTMYTGLCNFVERWDQLTLSQRKGLNYTYHLGCNCKIKSCYYLPCFVTSKNECLWTDMLSNFGYPGYQSKHYACIRQKGGYCSWYRGWAPPDKSIINATDP

SEQ ID NO: 99 - protein, 188 aa, Homo sapiens
  HuTIMP3(K45E, F57N, K94N, E96T, D110N, K112T, R138T)
CTCSPSHPQDAFCNSDIVIRAEVVGKKLVKEGPNGTLVYTIKQMKMYRGFTKMPHVQYIHTEASESLCGLNLTVNKYQYLLTGRVYNGTMYTGLCNFVERWDQLTLSQRKGLNYTYHLGCNCKIKSCYYLPCFVTSKNECLWTDMLSNFGYPGYQSKHYACIRQKGGYCSWYRGWAPPDKSIINATDP